European Patent Application EP 4 382 599 A2, published June 12, 2024. Title: PROBIOTIC COMPOSITIONS AND USES THEREOF. Applicant: The University of British Columbia. Application US 18/317,071, filed May 13, 2023. The sequence listing filed with the application follows.

SEQUENCE LISTING (73 sequences)

SEQ ID NO: 1 - DNA, 21 bp, synthetic construct
  misc_feature 1..21: note = Primer
  source 1..21: mol_type = other DNA
gagctcgaattctcatgtttg

SEQ ID NO: 2 - DNA, 21 bp, synthetic construct
  misc_feature 1..21: note = Primer
  source 1..21: mol_type = other DNA
ggatcctctagagtcgacctg

SEQ ID NO: 3 - DNA, 52 bp, synthetic construct
  misc_feature 1..52: note = Primer
  source 1..52: mol_type = other DNA
gcatgcctgcaggtcgactctagaggatccgttatatacgctcgatttttgc

SEQ ID NO: 4 - DNA, 51 bp, synthetic construct
  misc_feature 1..51: note = Primer
  source 1..51: mol_type = other DNA
ataagctgtcaaacatgagaattcgagctcttattcatggctcatacgttg

SEQ ID NO: 5 - DNA, 20 bp, synthetic construct
  misc_feature 1..20: note = Primer
  source 1..20: mol_type = other DNA
cgttatggactgcaacatgg

SEQ ID NO: 6 - DNA, 20 bp, synthetic construct
  misc_feature 1..20: note = Primer
  source 1..20: mol_type = other DNA
gcaaacggcctaaatacagc

SEQ ID NO: 7 - DNA, 60 bp, synthetic construct
  misc_feature 1..60: note = Primer
  source 1..60: mol_type = other DNA
tgccaagcttgcatgcctgcaggtcgactctagaggatccattccggggatccgtcgacc

SEQ ID NO: 8 - DNA, 60 bp, synthetic construct
  misc_feature 1..60: note = Primer
  source 1..60: mol_type = other DNA
ctgatcagtgataagctgtcaaacatgagaattcgagctctgtaggctggagctgcttcg

SEQ ID NO: 9 - DNA, 60 bp, synthetic construct
  misc_feature 1..60: note = Primer
  source 1..60: mol_type = other DNA
ccaattactaccagcttcagcactaccagcactaccaatcctctttcggtaataaatctt

SEQ ID NO: 10 - DNA, 60 bp, synthetic construct
  misc_feature 1..60: note = Primer
  source 1..60: mol_type = other DNA
gtgagcgcgcgtaatacgactcactatagggcggatccggtctatcctttatgggagaac

SEQ ID NO: 11 - DNA, 90 bp, synthetic construct
  misc_feature 1..90: note = Primer
  source 1..90: mol_type = other DNA
gtgctgaagctggtagtaattggagtcatccacaatttgaaaaaggtagtgctggtagtgctgctggtagtcacggttacgtatcggcag

SEQ ID NO: 12 - DNA, 60 bp, synthetic construct
  misc_feature 1..60: note = Primer
  source 1..60: mol_type = other DNA
aattcaccactaccagcagcactaccagcactaccaccgtcaaacttaacgtcaataacg

SEQ ID NO: 13 - DNA, 60 bp, synthetic construct
  misc_feature 1..60: note = Primer
  source 1..60: mol_type = other DNA
agtgctggtagtgctgctggtagtggtgaatttaaagttacctatagtggtagtgacagc

SEQ ID NO: 14 - DNA, 60 bp, synthetic construct
  misc_feature 1..60: note = Primer
  source 1..60: mol_type = other DNA
cgatatcaagcttatcgataccgtcgacctcgagaattcccgtcaagataatccgataag

SEQ ID NO: 15 - DNA, 28 bp, synthetic construct
  misc_feature 1..28: note = Primer
  source 1..28: mol_type = other DNA
gaattgggtaccgggccccccctcgagg

SEQ ID NO: 16 - DNA, 28 bp, synthetic construct
  misc_feature 1..28: note = Primer
  source 1..28: mol_type = other DNA
gccctatagtgagtcgtattacgcgcgc

SEQ ID NO: 17 - DNA, 22 bp, synthetic construct
  misc_feature 1..22: note = Primer
  source 1..22: mol_type = other DNA
aactgttggggttacttcggta

SEQ ID NO: 18 - DNA, 21 bp, synthetic construct
  misc_feature 1..21: note = Primer
  source 1..21: mol_type = other DNA
ctggttgttgctcaggtgttt

SEQ ID NO: 19 - protein, 485 aa, Vibrio cholerae
MKKQPKMTAIALILSGISGLAYGHGYVSAVENGVAEGRVTLCKFAANGTGEKNTHCGAIQYEPQSVEGPDGFPVTGPRDGKIASAESALAAALDEQTADRWVKRPIQAGPQTFEWTFTANHVTKDWKYYITKPNWNPNQPLSRDAFDLNPFCVVEGNMVQPPKRVSHECIVPEREGYQVILAVWDVGDTAASFYNVIDVKFDGNGPVLPDWNPAGQIIPSMDLSIGDTVYTRVFDNDGENPAYRTELKIDSETLTKANQWSYALATKINQTQKQQRAGQLNGDQFVPVYGTNPIYLKEGSGLKSVEIGYQIEAPQPEYSLTVSGLAKEYEIGEQPIQLDLTLEAQGEMSAELTVYNHHQKPLASWSQAMTDGELKSITLELSEAKAGHHMLVSRIKDRDGNLQDQQTLDFMLVEPQTPPTPGDYDFVFPNGLKEYVAGTKVLASDGAIYQCKPWPYSGYCQQWTSNATQYQPGTGSHWEMAWDKR

SEQ ID NO: 20 - protein, 180 aa, Vibrio cholerae
HGYVSAVENGVAEGRVTLCKFAANGTGEKNTHCGAIQYEPQSVEGPDGFPVTGPRDGKIASAESALAAALDEQTADRWVKRPIQAGPQTFEWTFTANHVTKDWKYYITKPNWNPNQPLSRDAFDLNPFCVVEGNMVQPPKRVSHECIVPEREGYQVILAVWDVGDTAASFYNVIDVKFDG

SEQ ID NO: 21 - protein, 1229 aa, Lactobacillus reuteri
MYLGGLIMLSRKNYKETIRKQTPTKQYYTIKKLTVGVTSVLIGLSFMGELEGDSVHADTMTASSESTSVTSTTAQDGLKKSPQLYLQVTDTNNPSTPLSASSTGTSKNVTSSAAVQVKSASDEEDSDSTLAKGENKFARSAVKDSVTDGKTSTAEINPAKLSSPALITQLNQSLAKSSTSDAAKANDELEIKATDPTNYPNCGDVYGPLFELDASGQLVNKDEVISLKDMYIFQILKLVNTKDSDFQYVILTMNRKDTADRSVYLFVTGSNYSNAVVVKVKPNDTYELSKTGYSVTYTEPTTINGHYVDGTFYVTGSTYDDGFIMPDWQLQHLQIIYSLGNYDPSNTDATSVCEIMPSYEKVPVIKYSGVPSNISQPKVYITGFTGQEFNVTDIINNYKKVFKGYYLQNPNVASMGTLSQFENGGYYLKTYYDNDGNVDFKGLYHQIDDQGTMSVSVLNADNKTIVGPENILAGKSHNFNFNGHNWIARNPYVTSSAHEVILKYAKLGSVIPVDENGNKINDGWQYVNDPDDASKATSPYEKAPVIDGYVAVNPDETIVLPHNLSSDTKIYYRKRIKVTYSGSDSKTYDGNPANFEPTTVQWSGLKGLNTSTLTSADFTWNTADKKAPTDAGKYTLSLNTTGEAALRKANPNYDLKTISGSYTYTINPLGIDKVTYSGSDSKTYDGNPANFEPTTVQWSGLKGLNTSTLTSADFTWNTADKKAPTDAGKYTLSLNTTGEAALRKANPNYDLKTISGSYTYTINPLGIDKVTYSGSDSKTYDGNPANFEPTTVQWSGLKGLNTSTLTSADFTWNTADKKAPTDAGKYTLSLNTTGEAALRKANPNYDLKTISGSYTYTINPLGIDKVTYSGSDSKTYDGNPANFEPTTVQWSGLKGLNTSTLTSADFTWNTADKKAPTDAGKYTLSLNTTGEAALRKANPNYDLKTISGSYTYTINPLGIDKVTYSGSDSKTYDGNPANFEPTTVQWSGLKGLNTSTLTSADFTWNTADKKAPTDAGKYTLSLNTTGEAALRKANPNYDLKTISGSYTYTINPLGIVTVNYKGYDKKVYDGQPGTINPGKLTWSKLPDGTSLKMPTWSIDDFAWETADGLAPTAVGTYRIILTDAGKAALKKINPNYDLSSITGVFTYEIKPAQTPEILGQTPEQQPGQNTNQSGAENGFGSSTRPNASTNSNLNQLPQTGNEHSNTALAGLALAFLTAMLGLGKKRKHD

SEQ ID NO: 22 - DNA, 540 bp, synthetic construct
  misc_feature 1..540: note = Harmonized Sequence
  source 1..540: mol_type = other DNA
cacggttacgtatcggcagttgaaaacggtgtagccgaagggcgtgtaactctttgtaaatttgcagccaacggtacaggggagaaaaacacacactgtggtgcaattcaatatgaacctcaatctgtagaaggtcctgatggtttccctgtaacaggtcctcgtgatggtaaaattgcctctgcagaatctgcccttgcagccgcacttgatgaacaaactgcagaccgttgggtcaagcgtcctattcaagcaggtcctcaaactttcgagtggaccttcactgcaaaccacgtaacgaaggattggaagtactacattactaagccaaactggaacccaaaccagcctcttagccgtgatgcatttgacttgaaccctttctgtgtcgtagaagggaacatggttcagcctcctaagcgtgtatctcacgaatgtattgttcctgaacgtgaagggtaccaggtaatcctagcagtctgggatgtaggtgatactgcagcctcgttctacaacgttattgacgttaagtttgacggt

SEQ ID NO: 23 - DNA, 3690 bp, Lactobacillus reuteri
  source 1..3690: mol_type = genomic DNA
ttgtatttaggagggttaataatgctatcaagaaaaaattataaggaaactatacgaaaacagacacctacaaaacagtactatactattaagaaattaactgttggggttacttcggtattaattggtctatcctttatgggagaactagaaggggatagcgttcatgcggacacgatgacagcaagcagtgagtcaacaagtgttacgtcgacgactgctcaggatggtttaaaaaaatctccacaactctatttgcaagttactgatacaaataacccaagtacaccattaagtgcttcatccacagggactagtaagaatgttacctcatcagctgcggtacaagtgaagtccgctagtgatgaagaagatagtgattctacactagctaagggagaaaataaatttgctcggtcagcagtaaaagattcagtcactgatgggaaaacaagtacagcagaaattaatccggcaaaattaagcagtcctgctttaataacgcaactcaaccaatccttagctaagagcagtacgagtgatgcagcaaaagctaatgatgagttagaaattaaagcaacagatccgactaattatccaaactgtggcgatgtgtatgggccattatttgaattggatgctagcggacagcttgttaataaagatgaagttatatctcttaaagatatgtatattttccaaatattgaaattagtaaatacaaaagatagtgactttcaatatgtaatattaacaatgaatcgtaaagatactgcagataggtctgtatatctttttgtaactggaagcaattatagtaatgctgttgttgttaaagtaaagccaaatgatacttatgaattaagtaaaactggatatagtgttacttatacagaaccaacaactataaatggacattatgttgatggaactttttatgttacaggaagtacttacgatgatggttttataatgccagattggcaactgcagcaccttcagattatatatagtttaggaaattatgatccaagcaatactgacgcaacatcagtttgtgaaataatgccaagttatgaaaaggtaccggtaattaaatatagtggagtaccttcaaatattagccaacctaaggtttacattaccgggtttacgggtcaagagtttaacgttacagatattattaacaattataagaaagtttttaagggctactatcttcaaaatcctaatgtggcgtccatgggaactctttcccaatttgagaatggtggttattacttaaagacatattatgataatgatggtaatgttgactttaagggcttgtatcatcaaattgatgatcagggaacaatgagtgtgagtgttcttaatgcagataataaaacaattgttggacctgaaaatattcttgctggtaaatcgcataactttaactttaatggtcataactggattgcgcggaatccttatgtcactagttcagctcacgaagtcatattaaagtatgctaagttaggttcagttattcctgttgatgaaaacggaaataaaataaacgatggatggcaatatgttaatgatccagatgatgcttccaaagccactagcccatatgaaaaagcgccagttatcgatggttatgtagctgtaaatccagatgaaacgatcgttcttcctcataacttaagtagtgacacaaagatttattaccgaaagaggattaaagttacctatagtggtagtgacagcaagacctacgatggtaacccagctaacttcgagccaacgacagttcagtggagtggcttgaaaggactgaacacttcaaccttaacgtccgctgacttcacgtggaatactgcggataagaaggcaccaacggatgccggtaagtacacacttagtttgaatacgaccggagaagcagccttacgtaaggctaacccgaactatgatctcaagacaattagcggtagttacacctacacgattaatccactagggattgataaagttacctatagtggtagtgacagcaagacctacgatggtaacccagctaacttcgagccaacgacagttcagtggagtggcttgaaaggactgaacacttcaaccttaacgtccgctgacttcacgtggaatactgcggataagaaggcaccaacggatgccggtaagtacacacttagtttgaatacgaccggagaagcagccttacgtaaggctaacccgaactatgatctcaagacaattagcggtagttacacctacacgattaatccactagggattgataaagttacctatagtggtagtgacagcaagacctacgatggtaacccagctaacttcgagccaacgacagttcagtggagtggcttgaaaggactgaacacttcaaccttaacgtccgctgacttcacgtggaatactgcggataagaaggcaccaacggatgccggtaagtacacacttagtttgaatacgaccggagaagcagccttacgtaaggctaacccgaactatgatctcaagacaattagcggtagttacacctacacgattaatccactagggattgataaagttacctatagtggtagtgacagcaagacctacgatggtaacccagctaacttcgagccaacgacagttcagtggagtggcttgaaaggactgaacacttcaaccttaacgtccgctgacttcacgtggaatactgcggataagaaggcaccaacggatgccggtaagtacacacttagtttgaatacgaccggagaagcagccttacgtaaggctaacccgaactatgatctcaagacaattagcggtagttacacctacacgattaatccactagggattgataaagttacctatagtggtagtgacagcaagacctacgatggtaacccagctaacttcgagccaacgacagttcagtggagtggcttgaaaggactgaacacttcaaccttaacgtccgctgacttcacgtggaatactgcggataagaaggcaccaacggatgccggtaagtacacacttagtttgaatacgaccggagaagcagccttacgtaaggctaacccgaactatgatctcaagacaattagcggtagttacacctacacgattaatccactagggattgtgactgtaaattacaagggctatgataagaaagtctatgatggtcaacctggaacgattaatccgggtaaattaacgtggagtaagttgccagatggtacttcattgaagatgccaacatggagtatagatgatttcgcttgggaaacagctgatggcttagcaccaacggcagtaggaacttatcggattatcttgacggatgctggtaaggctgcactaaagaagattaatccaaattatgacttaagcagtattactggtgtctttacttatgaaattaagccagcacagacaccagaaatcttaggccaaacacctgagcaacaaccaggccaaaatactaatcaatcaggagctgaaaacggctttggttcttctacaaggcctaatgcatcaactaactccaatcttaatcaacttccacagactggtaatgagcattctaatactgcacttgctggtctagcattggctttcttgactgctatgcttggtttgggcaagaagcgtaaacatgattag

SEQ ID NO: 24 - DNA, 4350 bp, synthetic construct
  misc_feature 1..4350: note = GbpA-MBP Chimeric Sequence
  source 1..4350: mol_type = other DNA
ttgtatttaggagggttaataatgctatcaagaaaaaattataaggaaactatacgaaaacagacacctacaaaacagtactatactattaagaaattaactgttggggttacttcggtattaattggtctatcctttatgggagaactagaaggggatagcgttcatgcggacacgatgacagcaagcagtgagtcaacaagtgttacgtcgacgactgctcaggatggtttaaaaaaatctccacaactctatttgcaagttactgatacaaataacccaagtacaccattaagtgcttcatccacagggactagtaagaatgttacctcatcagctgcggtacaagtgaagtccgctagtgatgaagaagatagtgattctacactagctaagggagaaaataaatttgctcggtcagcagtaaaagattcagtcactgatgggaaaacaagtacagcagaaattaatccggcaaaattaagcagtcctgctttaataacgcaactcaaccaatccttagctaagagcagtacgagtgatgcagcaaaagctaatgatgagttagaaattaaagcaacagatccgactaattatccaaactgtggcgatgtgtatgggccattatttgaattggatgctagcggacagcttgttaataaagatgaagttatatctcttaaagatatgtatattttccaaatattgaaattagtaaatacaaaagatagtgactttcaatatgtaatattaacaatgaatcgtaaagatactgcagataggtctgtatatctttttgtaactggaagcaattatagtaatgctgttgttgttaaagtaaagccaaatgatacttatgaattaagtaaaactggatatagtgttacttatacagaaccaacaactataaatggacattatgttgatggaactttttatgttacaggaagtacttacgatgatggttttataatgccagattggcaactgcagcaccttcagattatatatagtttaggaaattatgatccaagcaatactgacgcaacatcagtttgtgaaataatgccaagttatgaaaaggtaccggtaattaaatatagtggagtaccttcaaatattagccaacctaaggtttacattaccgggtttacgggtcaagagtttaacgttacagatattattaacaattataagaaagtttttaagggctactatcttcaaaatcctaatgtggcgtccatgggaactctttcccaatttgagaatggtggttattacttaaagacatattatgataatgatggtaatgttgactttaagggcttgtatcatcaaattgatgatcagggaacaatgagtgtgagtgttcttaatgcagataataaaacaattgttggacctgaaaatattcttgctggtaaatcgcataactttaactttaatggtcataactggattgcgcggaatccttatgtcactagttcagctcacgaagtcatattaaagtatgctaagttaggttcagttattcctgttgatgaaaacggaaataaaataaacgatggatggcaatatgttaatgatccagatgatgcttccaaagccactagcccatatgaaaaagcgccagttatcgatggttatgtagctgtaaatccagatgaaacgatcgttcttcctcataacttaagtagtgacacaaagatttattaccgaaagaggattggtagtgctggtagtgctgaagctggtagtaattggagtcatccacaatttgaaaaaggtagtgctggtagtgctgctggtagtcacggttacgtatcggcagttgaaaacggtgtagccgaagggcgtgtaactctttgtaaatttgcagccaacggtacaggggagaaaaacacacactgtggtgcaattcaatatgaacctcaatctgtagaaggtcctgatggtttccctgtaacaggtcctcgtgatggtaaaattgcctctgcagaatctgcccttgcagccgcacttgatgaacaaactgcagaccgttgggtcaagcgtcctattcaagcaggtcctcaaactttcgagtggaccttcactgcaaaccacgtaacgaaggattggaagtactacattactaagccaaactggaacccaaaccagcctcttagccgtgatgcatttgacttgaaccctttctgtgtcgtagaagggaacatggttcagcctcctaagcgtgtatctcacgaatgtattgttcctgaacgtgaagggtaccaggtaatcctagcagtctgggatgtaggtgatactgcagcctcgttctacaacgttattgacgttaagtttgacggtggtagtgctggtagtgctgctggtagtggtgaatttaaagttacctatagtggtagtgacagcaagacctacgatggtaacccagctaacttcgagccaacgacagttcagtggagtggcttgaaaggactgaacacttcaaccttaacgtccgctgacttcacgtggaatactgcggataagaaggcaccaacggatgccggtaagtacacacttagtttgaatacgaccggagaagcagccttacgtaaggctaacccgaactatgatctcaagacaattagcggtagttacacctacacgattaatccactagggattgataaagttacctatagtggtagtgacagcaagacctacgatggtaacccagctaacttcgagccaacgacagttcagtggagtggcttgaaaggactgaacacttcaaccttaacgtccgctgacttcacgtggaatactgcggataagaaggcaccaacggatgccggtaagtacacacttagtttgaatacgaccggagaagcagccttacgtaaggctaacccgaactatgatctcaagacaattagcggtagttacacctacacgattaatccactagggattgataaagttacctatagtggtagtgacagcaagacctacgatggtaacccagctaacttcgagccaacgacagttcagtggagtggcttgaaaggactgaacacttcaaccttaacgtccgctgacttcacgtggaatactgcggataagaaggcaccaacggatgccggtaagtacacacttagtttgaatacgaccggagaagcagccttacgtaaggctaacccgaactatgatctcaagacaattagcggtagttacacctacacgattaatccactagggattgataaagttacctatagtggtagtgacagcaagacctacgatggtaacccagctaacttcgagccaacgacagttcagtggagtggcttgaaaggactgaacacttcaaccttaacgtccgctgacttcacgtggaatactgcggataagaaggcaccaacggatgccggtaagtacacacttagtttgaatacgaccggagaagcagccttacgtaaggctaacccgaactatgatctcaagacaattagcggtagttacacctacacgattaatccactagggattgataaagttacctatagtggtagtgacagcaagacctacgatggtaacccagctaacttcgagccaacgacagttcagtggagtggcttgaaaggactgaacacttcaaccttaacgtccgctgacttcacgtggaatactgcggataagaaggcaccaacggatgccggtaagtacacacttagtttgaatacgaccggagaagcagccttacgtaaggctaacccgaactatgatctcaagacaattagcggtagttacacctacacgattaatccactagggattgtgactgtaaattacaagggctatgataagaaagtctatgatggtcaacctggaacgattaatccgggtaaattaacgtggagtaagttgccagatggtacttcattgaagatgccaacatggagtatagatgatttcgcttgggaaacagctgatggcttagcaccaacggcagtaggaacttatcggattatcttgacggatgctggtaaggctgcactaaagaagattaatccaaattatgacttaagcagtattactggtgtctttacttatgaaattaagccagcacagacaccagaaatcttaggccaaacacctgagcaacaaccaggccaaaatactaatcaatcaggagctgaaaacggctttggttcttctacaaggcctaatgcatcaactaactccaatcttaatcaacttccacagactggtaatgagcattctaatactgcacttgctggtctagcattggctttcttgactgctatgcttggtttgggcaagaagcgtaaacatgattag

SEQ ID NO: 25 - DNA, 7373 bp, Salmonella enterica
  source 1..7373: mol_type = genomic DNA
ttattcatggctcatacgttgttcgtattctggtctctggcgaggccattttttcgaaacgcctaatcagttccgccaggctaccggcctgcattttttccatgactctggcgcggtgcacctctacggtacgcaccgcgatattcatcgcttccgcaatttcacggttcataaatccttttgccaccaggctggccagctcacgctctttcggcgtcaactgctggtaacacagtataatctcacgacgcgccaccgctgccgatgaaaccgtcagcgcacgctccagcgccgcctgtagcggttttaccgataccggtttttgcagaaaatcgacggcgccgcgtttcatctgctccacggccatcggtacatcgccatgcccggtaagaaaaacaaccgccagggtacttccgcactggcgcaacgcatcatgaacgccctgcccatccagtaccggcattcgcatatccagtaatacgaccccggcctgatacagactggcctgcgccaaaaaatccgccccctgcgtccagcattttacgtcatatcccagactttccagtaaaaacgcgcacgcgttagtgaccgccgtatcatcatccagtagatgaattgtcgccatccctgcccccattttcatgtaagaaatgtatcgtaaccaccgttcccgacagaccgtccggcgcggtctggttcctgatgctgatatcgccccgcccataccgcaccagccgctggcaaatcgccagccctaagcccatcccctctttacgggtggtcataaacggctgaaacgcctgacgtaatagcgcctcatcgattcccccggcgttatcctgtaaaacaatactgatgccgttttcagtgcgttcagcaacgatccataaatgggtggcgcccgcctgagccgcattaagaatgatattcgccagcacctgttccagcagcactgacggcagcgttacgcgcagcgcagcgctaacctcggtatgcagagtcactgtcggaaactgttgcgccatacgcaacaattgccagacatgatcaatcgcctcgcgaatggctatggccttccacgcttcggttagcaccgggttgccctgcgcctggctgacccagtgacgcaggttacgcagagtatccgcaccgcgttgcgcctgctggtcaatctgctccagcgccggcagcaagggatgctgttcatctgcagcgcgcagtcgaatcaggcacccctgggcataatgtcgaatcgcggaaagcggctgattaagctcatgggcaaacccggaggtcatttcacccaacacgctcatttgccgggcggtttccagcgcccgctcatgctgatgaagaactacgctattacgttccagttgctttccacgtcgacgcaccagcagcatgacccaaatataattgagcgtgagcaacaagaacgccagaatcacgccgccgaccattagctggtgctggattaaccaacttttgacatccagccacagtcgacgctgctgagggtgctgacgaacatcacgcagcaaggcttccacctgactggtggacgcaggcgcgccccagtgaaatgacgcggcggcgggcgcgttgaatagcgctcgcgttacgcgatccgccagcgcatcgcttaccgcaggtagcgccgcgaacgaccagtcaggatataacggcgtactggttaagcaaggcaggggcgtcggtcgggaaagcagcgcgataaagtcctttttattaatcaatccttcctgatccatattttctaacaggcacactggcacaattgccgcctgcaccgctttttcgcgcagcatatagactaaggcatcgccaggaaatccggtaaaacggagatgaaaatcgcgctccgggcgtaagcccgcgtcgctgagcgctttatagcctaataaatagccgccaaacgcctgagcatcaatcgcgccgacggtcttaccgatgagatcatgcgccgtggtgatgccgctatcgcgccgggtcaaaatcacgctgccaataacattactcaccgctttcccatcgcgcgtggagcgcagggaagctaaccagcgcagcggcgcatggctgttcagttggacaaattgcgccgggttggttatcacaaactgcacggttccctggttaacggcctcctgcatttgatgcagatccagcggctggatgtgaaaggtttcgcctggaagctgttggcttaatgtctttgccaacggttgccagtggctacgcgtagacgcctcgccgcgcatggccaaaataccgatattccacgtccctgcccacgcgccatgacaaagtagccctactgccgccaacaccgccaggcgccttacggttttacctctcaccccaatatccctgtcaattatgttgttttagatcaacaacaagccgggtatgtggttaaccacaatagagcgcaccccgcctcgatttttacactgtaaatcatcgacattttttattcattacacatgaaccaacatcgtgacaaatgtttcattgttggcaatgtggacgggagtcaatatggacagcagtaaacggcaatttctccagcagcttggcgtcctgaccgctggcgcctcgctggttccgctggctgaagcgaaatttcctttttcgccggagcggcatgaaggctctccccgacaccgttacgccatgcttatcgatctgcggcgttgtatcggctgtcagtcctgtaccgtaagttgcactattgaaaaccaaacgccgcaaggcgcgtttcgtacgacggtgaaccaataccaggtccagcgtgaaggtagtcaggaagtcacgaatgtgctgttgccgcgtctgtgcaaccattgcgataaccccccctgtgtgccggtctgcccggtacaagccacctttcagcgggaagatggcattgtggtggtggataacaaacgctgcgtcggctgcgcctattgtgtccaggcgtgtccttacgacgcccgatttatcaatcatgaaacgcaaactgccgataaatgcacgttttgcgtccatcgtctggaagccggactgttacccgcttgcgtagagtcctgcgtcggcggcgcgcgtattattggcgatatcaaagatccccatagccgcatcgccaccatgcttcatcagcatcgcgacgctatcaaggtattaaagccggaaaacggcacgtcgccccatgttttctacctgggtctggacgacgcctttgtcaccccattaatgggccgtgcgcagcccgcgctttggcaggaggtctgaatgacgcattcactcatcattgaagaagtgctggctcacccgcaggacattagctggctgccgtgggcggtacaatatttcttttttattggcattgccgcctgcgccgcactgtttgcctgttatcttcactggcggaaaaaagacgccgcaacagaagaaaatcgggcattactgattgccattacctgtgcgattaccgcaccgctggcgctgacggcggatctgcaccagaccgcccgcgtctggcatttctatgcctggccgacgccctggtcgtggatgccctggggagcgttattcctgccgctgtttaccggatttctcgctctgtggttcctggcgcagcagattaaacgattattcaataaaagttacaacgtcactaaatggttggcgttagccagcgcgctttgcgcggtgggcctgttgatttataccggccgcgaagtctccgttgtgctggcgcgcccaatctggtttagctacgccttccccgtggcgatgtttcttagcgccttacaggcgttcttcgcgctgatgattgtcgccgcccgacgcgactcggtaaggctgccaaaaatattgtggggacaaatctggacgctggcggcgctggggctggttgtggccatgtgggttagcggcgatacgctttccggcacggcaatccgtcagtggattaccgtcgccctgtcagccaaatattacgctgtcggctgggtagcgctgtgggtatgcacactgctgttctgtagcctggcgctacgccatccgttatcacagctaagacgcgtcctgctggttctcagcgcgctggcgctatgttggctgatgcgctggacattgttgattcaggtacaaaccgtccccaagttcaacgcgcaatttaacccttactcgttaccaggcggaacggatggctggctggctattctcggcaccttcggcctgtggatagcgctactgattattattcgtgaaacgctgaacggactcaccaggagattacaacatggctaatttaacccgtcgtcagtggctaaaagtcggtctcgccgtcggtgggatggtcacttttggtctgagctaccgtgatgtggcgaaacgcgcaattgatggcctgttaaacgggacgtccggcaaggtaacgcgcgaccgcatctttggcaatgcgttaattccggaggcgcaggcgcaaacacactggcagcaaaatccacaacaaaccatcgccatgacgcaatgcttcggctgttggacacagtgcggtatccgcgcccgggttaatgccgatggcaaagtgatacgcatcgccggcaatccctatcaccccttgtcgcaggaacacccgattgactcgtccgtcccttttagcgaagccatggagcaactggcgggagaaagcggtcttgacgcccgctcaaccgcctgcgcgcgcggcgccacgctgctggaaagcctgtacagtccgctacgactgcttgaaccgatgaaacgcgtgggtaaacgcggcgaagggaaatggcagcgcatcagctttgagcaacttattgaagaagtcgtggaaggcggcgatctgtttggcgaaggtcatgtggacggactgcgcgctattcatgcgccggatacgccaattgacgcaaagcaccccagtttcgggcccaaaaccaatcagttactggtcacgaataccagcgacgaaggccgcgatgcgtttctgcgtcgttttgcgctaaatagcttcggcagcaagaatttcggcgcgcatggcgcctactgtggactggcttaccgggccggctccggggcattgatgggcgatctggataaaaacccgcatgtcaaacccgactgggaaaacgtggagtttgcgctctttatgggcacctccccggcacagtccggcaatccgtttaaacgccaggcacgtcagttggcgagcgcccgactgcgtgagaattttcaatacgtcgtggtcgcccccgccctccccttatcaacggtgctcgccgatcctcgcggtcgctggcaaccggtcatgcccggcagtgattcggcgctggcaatggggatgatccgctggatcatggataatcaacgttataatgctgattatctggcgattcccggcgtacaggcgatgcagcaggccggcgagcaaagttggaccaacgccacgcacctggtcattgcggatgagctgccgacgcttgccggacaacacctgacgctgcgccatcttacgcccgatggcgaagagacccctgtcgtactgaataccgacggcgagttggtcgatgcgtccacttgccgacaggcacggcttttcgtgacgcagtacgttacgctcgccgacggccaacgggtcacggtgaagagcgggttgcaacgcctgaaagaggcggcagaaaagctctcgttggcgcaatacagcgaacagtgcggcgtgccggaagcgcaaattatcgcgctggcggaaacctttaccagtcacggacgtaaagctgcggtcatcagtcacggcggcatgatggccggcaatgggttttataacgcctggtcggtcatgatgcttaacgcgctgatcggcaacctcagcttgtccggcggcgtctttgtcggcggcggcaaattcaacggcgttagcgacggcccccgctacaacatgaacagttttgccggaaaagtgaaaccgtccgggttaagtattgcccgtagcaaaaccgcttatgaagcatcggaagaataccgcgacaaaattgccggtgggcaatccccttatccagccaaagcgccgtggtatccctttgtggcaggccagcttaccgaactgttgacctccgcgctcgaaggctatccttatccgcttaaagcctggatttccaatatgagcaacccgttttacggtgttcccggtctacgcgccgtggcggaagaaaaactaaaagaccctcgccgactgccgctctttatcgcgattgacgcctttatgaatgaaacgacggcgctggcggattacattgtgccggatacgcacaattttgagagctggggctttacggcgccctggggcggcgtagccagtaaagccactaccgcccgctggccggttgtcgcccccgccactcaccgcacggcggacgggcaacctgtctcaatggaagcattttgtattgcggtagcaaaacggctccatctgcccggcttcggcgaccgggcgataaccgatccgcagggcaatacttttccactgaaccgggcggaagacttctatctgcgcgtagccgctaatatcgcctttatgggcaagacgccggtcgcgctggcaaatcaggaagatatttcgcttaccggcgtcagccgcattctgccagcaattcagcacacgcttaaagctgatgaggtcggtcgcgtggcgtttatctactcgcgtggcggccggtttgcgcccgaggatagcggctatacggagcaacggttaggtaacgcgtggaaaaaacccttacagatctggaatgcagatgtcgccgcccaccgtcacgccatcaccggggagcgcttcagcggttgcccggtctggtatccggcgcgtttgtcagatggtcgtgcgattgacgaccagtttcccattgggcaatggccgctgaaactgatttcatttaaatcaaataccatgtccagctcaacagccgtcatcccgcgcttacaccatgtgaagccagcaaacctggtggcgctgaatccgcaagacggcgagcgttatggactgcaacatggcgatcgggtacggatcattacgccgggcggtcaggtcgtggcgcaaatcagtttgttaaatggcgtgatgccaggcgtcatcgccatcgaacacggatatggccaccgcgagatgggcgcaacgcagcactctctggatggcgtgcctatgccgtatgatccacaaatcagggcaggcataaatcttaacgatctgggctttgccgatccgacaagaaccattaccaacacctggctcgactgggtttctggcgcggcagtacgtcaggggctgccggcaaaaatcgagcgtatataac

SEQ ID NO: 26 - DNA, 1458 bp, Vibrio cholerae
  source 1..1458: mol_type = genomic DNA
atgaaaaaacaacctaaaatgaccgctattgccctgatcctctctggtatcagtggattagcgtatggacacggctacgtttccgcagtggaaaacggtgtcgccgaaggacgtgtcaccttgtgtaaatttgccgctaacggcactggagagaaaaacactcactgtggcgcgattcaatacgaaccacaaagtgtcgaaggcccagatggcttcccggtcactggccctcgtgatggcaaaattgccagtgcggaatcggcactggcggcagcgctggatgagcaaaccgccgaccgttgggtaaagcgcccaattcaagctggcccacaaaccttcgagtggacgttcaccgccaaccacgtcacaaaggattggaaatactacattaccaaaccaaactggaacccaaaccagccattgtcgcgtgatgcatttgacctcaatccgttctgtgtcgttgaaggaaatatggtgcagccaccaaaacgtgtcagccacgaatgtatcgtgcctgagcgcgaagggtatcaggtcatcctcgccgtatgggatgttggcgataccgcagcttccttctacaacgtgatcgacgtgaaatttgacggtaacggcccagtgttacccgattggaacccagcaggtcaaatcattccaagtatggatctcagcattggcgataccgtgtacactcgcgtgtttgataacgatggggaaaaccctgcttatcgcactgagctaaaaattgactctgagacgctaaccaaagccaatcaatggtcttacgctctggcgactaaaattaaccaaacgcaaaaacagcaacgtgctggtcagcttaatggcgatcaatttgttcccgtttacggcaccaacccgatttatctgaaagaaggcagtggcttgaagagtgttgaaattggctaccaaattgaagcgccacagcctgagtattcactgacggtttctggtctagcgaaagagtatgagattggcgaacaaccgattcagcttgacctgactttagaagcgcaaggtgaaatgagcgcagagctgaccgtgtataaccaccaccaaaaaccgctggcaagttggtcacaagcgatgacggatggcgagctgaaatccatcacgctagagctgagcgaagctaaagcgggacatcatatgttggtttctcgcatcaaagatcgcgatggcaatctgcaagatcaacaaactctcgatttcatgctggttgaaccgcaaacaccaccaacaccgggtgactacgactttgtgttcccgaatggcctgaaagagtacgtggctggcaccaaagtgctcgctagtgatggcgcaatctaccaatgtaagccatggccatactctggctactgccagcaatggacaagtaacgctactcaataccaaccgggtactggcagtcattgggaaatggcgtgggataaacgttaa

SEQ ID NO: 27 - DNA, 540 bp, Vibrio cholerae
  source 1..540: mol_type = genomic DNA
atgaaaaaacaacctaaaatgaccgctattgccctgatcctctctggtatcagtggattagcgtatggacacggctacgtttccgcagtggaaaacggtgtcgccgaaggacgtgtcaccttgtgtaaatttgccgctaacggcactggagagaaaaacactcactgtggcgcgattcaatacgaaccacaaagtgtcgaaggcccagatggcttcccggtcactggccctcgtgatggcaaaattgccagtgcggaatcggcactggcggcagcgctggatgagcaaaccgccgaccgttgggtaaagcgcccaattcaagctggcccacaaaccttcgagtggacgttcaccgccaaccacgtcacaaaggattggaaatactacattaccaaaccaaactggaacccaaaccagccattgtcgcgtgatgcatttgacctcaatccgttctgtgtcgttgaaggaaatatggtgcagccaccaaaacgtgtcagccacgaatgtatcgtgcctgagcgcgaagggtatcaggtcatc

SEQ ID NO: 28 - protein, 1222 aa, Lactobacillus reuteri
MLSRKNYKETIRKQTPTKQYYTIKKLTVGVTSVLIGLSFMGELEGDSVHADTMTASSESTSVTSTTAQDGLKKSPQLYLQVTDTNNPSTPLSASSTGTSKNVTSSAAVQVKSASDEEDSDSTLAKGENKFARSAVKDSVTDGKTSTAEINPAKLSSPALITQLNQSLAKSSTSDAAKANDELEIKATDPTNYPNCGDVYGPLFELDASGQLVNKDEVISLKDMYIFQILKLVNTKDSDFQYVILTMNRKDTADRSVYLFVTGSNYSNAVVVKVKPNDTYELSKTGYSVTYTEPTTINGHYVDGTFYVTGSTYDDGFIMPDWQLQHLQIIYSLGNYDPSNTDATSVCEIMPSYEKVPVIKYSGVPSNISQPKVYITGFTGQEFNVTDIINNYKKVFKGYYLQNPNVASMGTLSQFENGGYYLKTYYDNDGNVDFKGLYHQIDDQGTMSVSVLNADNKTIVGPENILAGKSHNFNFNGHNWIARNPYVTSSAHEVILKYAKLGSVIPVDENGNKINDGWQYVNDPDDASKATSPYEKAPVIDGYVAVNPDETIVLPHNLSSDTKIYYRKRIKVTYSGSDSKTYDGNPANFEPTTVQWSGLKGLNTSTLTSADFTWNTADKKAPTDAGKYTLSLNTTGEAALRKANPNYDLKTISGSYTYTINPLGIDKVTYSGSDSKTYDGNPANFEPTTVQWSGLKGLNTSTLTSADFTWNTADKKAPTDAGKYTLSLNTTGEAALRKANPNYDLKTISGSYTYTINPLGIDKVTYSGSDSKTYDGNPANFEPTTVQWSGLKGLNTSTLTSADFTWNTADKKAPTDAGKYTLSLNTTGEAALRKANPNYDLKTISGSYTYTINPLGIDKVTYSGSDSKTYDGNPANFEPTTVQWSGLKGLNTSTLTSADFTWNTADKKAPTDAGKYTLSLNTTGEAALRKANPNYDLKTISGSYTYTINPLGIDKVTYSGSDSKTYDGNPANFEPTTVQWSGLKGLNTSTLTSADFTWNTADKKAPTDAGKYTLSLNTTGEAALRKANPNYDLKTISGSYTYTINPLGIVTVNYKGYDKKVYDGQPGTINPGKLTWSKLPDGTSLKMPTWSIDDFAWETADGLAPTAVGTYRIILTDAGKAALKKINPNYDLSSITGVFTYEIKPAQTPEILGQTPEQQPGQNTNQSGAENGFGSSTRPNASTNSNLNQLPQTGNEHSNTALAGLALAFLTAMLGLGKKRKHD

SEQ ID NO: 29 - protein, 1442 aa, synthetic construct
  REGION 1..1442: note = GbpA-MBP Chimeric Sequence
MLSRKNYKETIRKQTPTKQYYTIKKLTVGVTSVLIGLSFMGELEGDSVHADTMTASSESTSVTSTTAQDGLKKSPQLYLQVTDTNNPSTPLSASSTGTSKNVTSSAAVQVKSASDEEDSDSTLAKGENKFARSAVKDSVTDGKTSTAEINPAKLSSPALITQLNQSLAKSSTSDAAKANDELEIKATDPTNYPNCGDVYGPLFELDASGQLVNKDEVISLKDMYIFQILKLVNTKDSDFQYVILTMNRKDTADRSVYLFVTGSNYSNAVVVKVKPNDTYELSKTGYSVTYTEPTTINGHYVDGTFYVTGSTYDDGFIMPDWQLQHLQIIYSLGNYDPSNTDATSVCEIMPSYEKVPVIKYSGVPSNISQPKVYITGFTGQEFNVTDIINNYKKVFKGYYLQNPNVASMGTLSQFENGGYYLKTYYDNDGNVDFKGLYHQIDDQGTMSVSVLNADNKTIVGPENILAGKSHNFNFNGHNWIARNPYVTSSAHEVILKYAKLGSVIPVDENGNKINDGWQYVNDPDDASKATSPYEKAPVIDGYVAVNPDETIVLPHNLSSDTKIYYRKRIGSAGSAEAGSNWSHPQFEKGSAGSAAGSHGYVSAVENGVAEGRVTLCKFAANGTGEKNTHCGAIQYEPQSVEGPDGFPVTGPRDGKIASAESALAAALDEQTADRWVKRPIQAGPQTFEWTFTANHVTKDWKYYITKPNWNPNQPLSRDAFDLNPFCVVEGNMVQPPKRVSHECIVPEREGYQVILAVWDVGDTAASFYNVIDVKFDGGSAGSAAGSGEFKVTYSGSDSKTYDGNPANFEPTTVQWSGLKGLNTSTLTSADFTWNTADKKAPTDAGKYTLSLNTTGEAALRKANPNYDLKTISGSYTYTINPLGIDKVTYSGSDSKTYDGNPANFEPTTVQWSGLKGLNTSTLTSADFTWNTADKKAPTDAGKYTLSLNTTGEAALRKANPNYDLKTISGSYTYTINPLGIDKVTYSGSDSKTYDGNPANFEPTTVQWSGLKGLNTSTLTSADFTWNTADKKAPTDAGKYTLSLNTTGEAALRKANPNYDLKTISGSYTYTINPLGIDKVTYSGSDSKTYDGNPANFEPTTVQWSGLKGLNTSTLTSADFTWNTADKKAPTDAGKYTLSLNTTGEAALRKANPNYDLKTISGSYTYTINPLGIDKVTYSGSDSKTYDGNPANFEPTTVQWSGLKGLNTSTLTSADFTWNTADKKAPTDAGKYTLSLNTTGEAALRKANPNYDLKTISGSYTYTINPLGIVTVNYKGYDKKVYDGQPGTINPGKLTWSKLPDGTSLKMPTWSIDDFAWETADGLAPTAVGTYRIILTDAGKAALKKINPNYDLSSITGVFTYEIKPAQTPEILGQTPEQQPGQNTNQSGAENGFGSSTRPNASTNSNLNQLPQTGNEHSNTALAGLALAFLTAMLGLGKKRKHD

SEQ ID NO: 30 - DNA, 4329 bp, synthetic construct
  misc_feature 1..4329: note = GbpA-MBP Chimeric Sequence
  source 1..4329: mol_type = other DNA
atgctatcaagaaaaaattataaggaaactatacgaaaacagacacctacaaaacagtactatactattaagaaattaactgttggggttacttcggtattaattggtctatcctttatgggagaactagaaggggatagcgttcatgcggacacgatgacagcaagcagtgagtcaacaagtgttacgtcgacgactgctcaggatggtttaaaaaaatctccacaactctatttgcaagttactgatacaaataacccaagtacaccattaagtgcttcatccacagggactagtaagaatgttacctcatcagctgcggtacaagtgaagtccgctagtgatgaagaagatagtgattctacactagctaagggagaaaataaatttgctcggtcagcagtaaaagattcagtcactgatgggaaaacaagtacagcagaaattaatccggcaaaattaagcagtcctgctttaataacgcaactcaaccaatccttagctaagagcagtacgagtgatgcagcaaaagctaatgatgagttagaaattaaagcaacagatccgactaattatccaaactgtggcgatgtgtatgggccattatttgaattggatgctagcggacagcttgttaataaagatgaagttatatctcttaaagatatgtatattttccaaatattgaaattagtaaatacaaaagatagtgactttcaatatgtaatattaacaatgaatcgtaaagatactgcagataggtctgtatatctttttgtaactggaagcaattatagtaatgctgttgttgttaaagtaaagccaaatgatacttatgaattaagtaaaactggatatagtgttacttatacagaaccaacaactataaatggacattatgttgatggaactttttatgttacaggaagtacttacgatgatggttttataatgccagattggcaactgcagcaccttcagattatatatagtttaggaaattatgatccaagcaatactgacgcaacatcagtttgtgaaataatgccaagttatgaaaaggtaccggtaattaaatatagtggagtaccttcaaatattagccaacctaaggtttacattaccgggtttacgggtcaagagtttaacgttacagatattattaacaattataagaaagtttttaagggctactatcttcaaaatcctaatgtggcgtccatgggaactctttcccaatttgagaatggtggttattacttaaagacatattatgataatgatggtaatgttgactttaagggcttgtatcatcaaattgatgatcagggaacaatgagtgtgagtgttcttaatgcagataataaaacaattgttggacctgaaaatattcttgctggtaaatcgcataactttaactttaatggtcataactggattgcgcggaatccttatgtcactagttcagctcacgaagtcatattaaagtatgctaagttaggttcagttattcctgttgatgaaaacggaaataaaataaacgatggatggcaatatgttaatgatccagatgatgcttccaaagccactagcccatatgaaaaagcgccagttatcgatggttatgtagctgtaaatccagatgaaacgatcgttcttcctcataacttaagtagtgacacaaagatttattaccgaaagaggattggtagtgctggtagtgctgaagctggtagtaattggagtcatccacaatttgaaaaaggtagtgctggtagtgctgctggtagtcacggttacgtatcggcagttgaaaacggtgtagccgaagggcgtgtaactctttgtaaatttgcagccaacggtacaggggagaaaaacacacactgtggtgcaattcaatatgaacctcaatctgtagaaggtcctgatggtttccctgtaacaggtcctcgtgatggtaaaattgcctctgcagaatctgcccttgcagccgcacttgatgaacaaactgcagaccgttgggtcaagcgtcctattcaagcaggtcctcaaactttcgagtggaccttcactgcaaaccacgtaacgaaggattggaagtactacattactaagccaaactggaacccaaaccagcctcttagccgtgatgcatttgacttgaaccctttctgtgtcgtagaagggaacatggttcagcctcctaagcgtgtatctcacgaatgtattgttcctgaacgtgaagggtaccaggtaatcctagcagtctgggatgtaggtgatactgcagcctcgttctacaacgttattgacgttaagtttgacggtggtagtgctggtagtgctgctggtagtggtgaatttaaagttacctatagtggtagtgacagcaagacctacgatggtaacccagctaacttcgagccaacgacagttcagtggagtggcttgaaaggactgaacacttcaaccttaacgtccgctgacttcacgtggaatactgcggataagaaggcaccaacggatgccggtaagtacacacttagtttgaatacgaccggagaagcagccttacgtaaggctaacccgaactatgatctcaagacaattagcggtagttacacctacacgattaatccactagggattgataaagttacctatagtggtagtgacagcaagacctacgatggtaacccagctaacttcgagccaacgacagttcagtggagtggcttgaaaggactgaacacttcaaccttaacgtccgctgacttcacgtggaatactgcggataagaaggcaccaacggatgccggtaagtacacacttagtttgaatacgaccggagaagcagccttacgtaaggctaacccgaactatgatctcaagacaattagcggtagttacacctacacgattaatccactagggattgataaagttacctatagtggtagtgacagcaagacctacgatggtaacccagctaacttcgagccaacgacagttcagtggagtggcttgaaaggactgaacacttcaaccttaacgtccgctgacttcacgtggaatactgcggataagaaggcaccaacggatgccggtaagtacacacttagtttgaatacgaccggagaagcagccttacgtaaggctaacccgaactatgatctcaagacaattagcggtagttacacctacacgattaatccactagggattgataaagttacctatagtggtagtgacagcaagacctacgatggtaacccagctaacttcgagccaacgacagttcagtggagtggcttgaaaggactgaacacttcaaccttaacgtccgctgacttcacgtggaatactgcggataagaaggcaccaacggatgccggtaagtacacacttagtttgaatacgaccggagaagcagccttacgtaaggctaacccgaactatgatctcaagacaattagcggtagttacacctacacgattaatccactagggattgataaagttacctatagtggtagtgacagcaagacctacgatggtaacccagctaacttcgagccaacgacagttcagtggagtggcttgaaaggactgaacacttcaaccttaacgtccgctgacttcacgtggaatactgcggataagaaggcaccaacggatgccggtaagtacacacttagtttgaatacgaccggagaagcagccttacgtaaggctaacccgaactatgatctcaagacaattagcggtagttacacctacacgattaatccactagggattgtgactgtaaattacaagggctatgataagaaagtctatgatggtcaacctggaacgattaatccgggtaaattaacgtggagtaagttgccagatggtacttcattgaagatgccaacatggagtatagatgatttcgcttgggaaacagctgatggcttagcaccaacggcagtaggaacttatcggattatcttgacggatgctggtaaggctgcactaaagaagattaatccaaattatgacttaagcagtattactggtgtctttacttatgaaattaagccagcacagacaccagaaatcttaggccaaacacctgagcaacaaccaggccaaaatactaatcaatcaggagctgaaaacggctttggttcttctacaaggcctaatgcatcaactaactccaatcttaatcaacttccacagactggtaatgagcattctaatactgcacttgctggtctagcattggctttcttgactgctatgcttggtttgggcaagaagcgtaaacatgattag

SEQ ID NO: 31 - DNA, 4991 bp, Salmonella enterica
  source 1..4991: mol_type = genomic DNA
cccaatatccctgtcaattatgttgttttagatcaacaacaagccgggtatgtggttaaccacaatagagcgcaccccgcctcgatttttacactgtaaatcatcgacattttttattcattacacatgaaccaacatcgtgacaaatgtttcattgttggcaatgtggacgggagtcaatatggacagcagtaaacggcaatttctccagcagcttggcgtcctgaccgctggcgcctcgctggttccgctggctgaagcgaaatttcctttttcgccggagcggcatgaaggctctccccgacaccgttacgccatgcttatcgatctgcggcgttgtatcggctgtcagtcctgtaccgtaagttgcactattgaaaaccaaacgccgcaaggcgcgtttcgtacgacggtgaaccaataccaggtccagcgtgaaggtagtcaggaagtcacgaatgtgctgttgccgcgtctgtgcaaccattgcgataaccccccctgtgtgccggtctgcccggtacaagccacctttcagcgggaagatggcattgtggtggtggataacaaacgctgcgtcggctgcgcctattgtgtccaggcgtgtccttacgacgcccgatttatcaatcatgaaacgcaaactgccgataaatgcacgttttgcgtccatcgtctggaagccggactgttacccgcttgcgtagagtcctgcgtcggcggcgcgcgtattattggcgatatcaaagatccccatagccgcatcgccaccatgcttcatcagcatcgcgacgctatcaaggtattaaagccggaaaacggcacgtcgccccatgttttctacctgggtctggacgacgcctttgtcaccccattaatgggccgtgcgcagcccgcgctttggcaggaggtctgaatgacgcattcactcatcattgaagaagtgctggctcacccgcaggacattagctggctgccgtgggcggtacaatatttcttttttattggcattgccgcctgcgccgcactgtttgcctgttatcttcactggcggaaaaaagacgccgcaacagaagaaaatcgggcattactgattgccattacctgtgcgattaccgcaccgctggcgctgacggcggatctgcaccagaccgcccgcgtctggcatttctatgcctggccgacgccctggtcgtggatgccctggggagcgttattcctgccgctgtttaccggatttctcgctctgtggttcctggcgcagcagattaaacgattattcaataaaagttacaacgtcactaaatggttggcgttagccagcgcgctttgcgcggtgggcctgttgatttataccggccgcgaagtctccgttgtgctggcgcgcccaatctggtttagctacgccttccccgtggcgatgtttcttagcgccttacaggcgttcttcgcgctgatgattgtcgccgcccgacgcgactcggtaaggctgccaaaaatattgtggggacaaatctggacgctggcggcgctggggctggttgtggccatgtgggttagcggcgatacgctttccggcacggcaatccgtcagtggattaccgtcgccctgtcagccaaatattacgctgtcggctgggtagcgctgtgggtatgcacactgctgttctgtagcctggcgctacgccatccgttatcacagctaagacgcgtcctgctggttctcagcgcgctggcgctatgttggctgatgcgctggacattgttgattcaggtacaaaccgtccccaagttcaacgcgcaatttaacccttactcgttaccaggcggaacggatggctggctggctattctcggcaccttcggcctgtggatagcgctactgattattattcgtgaaacgctgaacggactcaccaggagattacaacatggctaatttaacccgtcgtcagtggctaaaagtcggtctcgccgtcggtgggatggtcacttttggtctgagctaccgtgatgtggcgaaacgcgcaattgatggcctgttaaacgggacgtccggcaaggtaacgcgcgaccgcatctttggcaatgcgttaattccggaggcgcaggcgcaaacacactggcagcaaaatccacaacaaaccatcgccatgacgcaatgcttcggctgttggacacagtgcggtatccgcgcccgggttaatgccgatggcaaagtgatacgcatcgccggcaatccctatcaccccttgtcgcaggaacacccgattgactcgtccgtcccttttagcgaagccatggagcaactggcgggagaaagcggtcttgacgcccgctcaaccgcctgcgcgcgcggcgccacgctgctggaaagcctgtacagtccgctacgactgcttgaaccgatgaaacgcgtgggtaaacgcggcgaagggaaatggcagcgcatcagctttgagcaacttattgaagaagtcgtggaaggcggcgatctgtttggcgaaggtcatgtggacggactgcgcgctattcatgcgccggatacgccaattgacgcaaagcaccccagtttcgggcccaaaaccaatcagttactggtcacgaataccagcgacgaaggccgcgatgcgtttctgcgtcgttttgcgctaaatagcttcggcagcaagaatttcggcgcgcatggcgcctactgtggactggcttaccgggccggctccggggcattgatgggcgatctggataaaaacccgcatgtcaaacccgactgggaaaacgtggagtttgcgctctttatgggcacctccccggcacagtccggcaatccgtttaaacgccaggcacgtcagttggcgagcgcccgactgcgtgagaattttcaatacgtcgtggtcgcccccgccctccccttatcaacggtgctcgccgatcctcgcggtcgctggcaaccggtcatgcccggcagtgattcggcgctggcaatggggatgatccgctggatcatggataatcaacgttataatgctgattatctggcgattcccggcgtacaggcgatgcagcaggccggcgagcaaagttggaccaacgccacgcacctggtcattgcggatgagctgccgacgcttgccggacaacacctgacgctgcgccatcttacgcccgatggcgaagagacccctgtcgtactgaataccgacggcgagttggtcgatgcgtccacttgccgacaggcacggcttttcgtgacgcagtacgttacgctcgccgacggccaacgggtcacggtgaagagcgggttgcaacgcctgaaagaggcggcagaaaagctctcgttggcgcaatacagcgaacagtgcggcgtgccggaagcgcaaattatcgcgctggcggaaacctttaccagtcacggacgtaaagctgcggtcatcagtcacggcggcatgatggccggcaatgggttttataacgcctggtcggtcatgatgcttaacgcgctgatcggcaacctcagcttgtccggcggcgtctttgtcggcggcggcaaattcaacggcgttagcgacggcccccgctacaacatgaacagttttgccggaaaagtgaaaccgtccgggttaagtattgcccgtagcaaaaccgcttatgaagcatcggaagaataccgcgacaaaattgccggtgggcaatccccttatccagccaaagcgccgtggtatccctttgtggcaggccagcttaccgaactgttgacctccgcgctcgaaggctatccttatccgcttaaagcctggatttccaatatgagcaacccgttttacggtgttcccggtctacgcgccgtggcggaagaaaaactaaaagaccctcgccgactgccgctctttatcgcgattgacgcctttatgaatgaaacgacggcgctggcggattacattgtgccggatacgcacaattttgagagctggggctttacggcgccctggggcggcgtagccagtaaagccactaccgcccgctggccggttgtcgcccccgccactcaccgcacggcggacgggcaacctgtctcaatggaagcattttgtattgcggtagcaaaacggctccatctgcccggcttcggcgaccgggcgataaccgatccgcagggcaatacttttccactgaaccgggcggaagacttctatctgcgcgtagccgctaatatcgcctttatgggcaagacgccggtcgcgctggcaaatcaggaagatatttcgcttaccggcgtcagccgcattctgccagcaattcagcacacgcttaaagctgatgaggtcggtcgcgtggcgtttatctactcgcgtggcggccggtttgcgcccgaggatagcggctatacggagcaacggttaggtaacgcgtggaaaaaacccttacagatctggaatgcagatgtcgccgcccaccgtcacgccatcaccggggagcgcttcagcggttgcccggtctggtatccggcgcgtttgtcagatggtcgtgcgattgacgaccagtttcccattgggcaatggccgctgaaactgatttcatttaaatcaaataccatgtccagctcaacagccgtcatcccgcgcttacaccatgtgaagccagcaaacctggtggcgctgaatccgcaagacggcgagcgttatggactgcaacatggcgatcgggtacggatcattacgccgggcggtcaggtcgtggcgcaaatcagtttgttaaatggcgtgatgccaggcgtcatcgccatcgaacacggatatggccaccgcgagatgggcgcaacgcagcactctctggatggcgtgcctatgccgtatgatccacaaatcagggcaggcataaatcttaacgatctgggctttgccgatccgacaagaaccattaccaacacctggctcgactgggtttctggcgcggcagtacgtcaggggctgccggcaaaaatcgagcgtata

SEQ ID NO: 32 - DNA, 2374 bp, Salmonella enterica
  source 1..2374: mol_type = genomic DNA
tcatggctcatacgttgttcgtattctggtctctggcgaggccattttttcgaaacgcctaatcagttccgccaggctaccggcctgcattttttccatgactctggcgcggtgcacctctacggtacgcaccgcgatattcatcgcttccgcaatttcacggttcataaatccttttgccaccaggctggccagctcacgctctttcggcgtcaactgctggtaacacagtataatctcacgacgcgccaccgctgccgatgaaaccgtcagcgcacgctccagcgccgcctgtagcggttttaccgataccggtttttgcagaaaatcgacggcgccgcgtttcatctgctccacggccatcggtacatcgccatgcccggtaagaaaaacaaccgccagggtacttccgcactggcgcaacgcatcatgaacgccctgcccatccagtaccggcattcgcatatccagtaatacgaccccggcctgatacagactggcctgcgccaaaaaatccgccccctgcgtccagcattttacgtcatatcccagactttccagtaaaaacgcgcacgcgttagtgaccgccgtatcatcatccagtagatgaattgtcgccatccctgcccccattttcatgtaagaaatgtatcgtaaccaccgttcccgacagaccgtccggcgcggtctggttcctgatgctgatatcgccccgcccataccgcaccagccgctggcaaatcgccagccctaagcccatcccctctttacgggtggtcataaacggctgaaacgcctgacgtaatagcgcctcatcgattcccccggcgttatcctgtaaaacaatactgatgccgttttcagtgcgttcagcaacgatccataaatgggtggcgcccgcctgagccgcattaagaatgatattcgccagcacctgttccagcagcactgacggcagcgttacgcgcagcgcagcgctaacctcggtatgcagagtcactgtcggaaactgttgcgccatacgcaacaattgccagacatgatcaatcgcctcgcgaatggctatggccttccacgcttcggttagcaccgggttgccctgcgcctggctgacccagtgacgcaggttacgcagagtatccgcaccgcgttgcgcctgctggtcaatctgctccagcgccggcagcaagggatgctgttcatctgcagcgcgcagtcgaatcaggcacccctgggcataatgtcgaatcgcggaaagcggctgattaagctcatgggcaaacccggaggtcatttcacccaacacgctcatttgccgggcggtttccagcgcccgctcatgctgatgaagaactacgctattacgttccagttgctttccacgtcgacgcaccagcagcatgacccaaatataattgagcgtgagcaacaagaacgccagaatcacgccgccgaccattagctggtgctggattaaccaacttttgacatccagccacagtcgacgctgctgagggtgctgacgaacatcacgcagcaaggcttccacctgactggtggacgcaggcgcgccccagtgaaatgacgcggcggcgggcgcgttgaatagcgctcgcgttacgcgatccgccagcgcatcgcttaccgcaggtagcgccgcgaacgaccagtcaggatataacggcgtactggttaagcaaggcaggggcgtcggtcgggaaagcagcgcgataaagtcctttttattaatcaatccttcctgatccatattttctaacaggcacactggcacaattgccgcctgcaccgctttttcgcgcagcatatagactaaggcatcgccaggaaatccggtaaaacggagatgaaaatcgcgctccgggcgtaagcccgcgtcgctgagcgctttatagcctaataaatagccgccaaacgcctgagcatcaatcgcgccgacggtcttaccgatgagatcatgcgccgtggtgatgccgctatcgcgccgggtcaaaatcacgctgccaataacattactcaccgctttcccatcgcgcgtggagcgcagggaagctaaccagcgcagcggcgcatggctgttcagttggacaaattgcgccgggttggttatcacaaactgcacggttccctggttaacggcctcctgcatttgatgcagatccagcggctggatgtgaaaggtttcgcctggaagctgttggcttaatgtctttgccaacggttgccagtggctacgcgtagacgcctcgccgcgcatggccaaaataccgatattccacgtccctgcccacgcgccatgacaaagtagccctactgccgccaacaccgccaggcgccttacggttttacctctcac

SEQ ID NO: 33 - DNA, 3060 bp, Salmonella enterica
  source 1..3060: mol_type = genomic DNA
atggctaatttaacccgtcgtcagtggctaaaagtcggtctcgccgtcggtgggatggtcacttttggtctgagctaccgtgatgtggcgaaacgcgcaattgatggcctgttaaacgggacgtccggcaaggtaacgcgcgaccgcatctttggcaatgcgttaattccggaggcgcaggcgcaaacacactggcagcaaaatccacaacaaaccatcgccatgacgcaatgcttcggctgttggacacagtgcggtatccgcgcccgggttaatgccgatggcaaagtgatacgcatcgccggcaatccctatcaccccttgtcgcaggaacacccgattgactcgtccgtcccttttagcgaagccatggagcaactggcgggagaaagcggtcttgacgcccgctcaaccgcctgcgcgcgcggcgccacgctgctggaaagcctgtacagtccgctacgactgcttgaaccgatgaaacgcgtgggtaaacgcggcgaagggaaatggcagcgcatcagctttgagcaacttattgaagaagtcgtggaaggcggcgatctgtttggcgaaggtcatgtggacggactgcgcgctattcatgcgccggatacgccaattgacgcaaagcaccccagtttcgggcccaaaaccaatcagttactggtcacgaataccagcgacgaaggccgcgatgcgtttctgcgtcgttttgcgctaaatagcttcggcagcaagaatttcggcgcgcatggcgcctactgtggactggcttaccgggccggctccggggcattgatgggcgatctggataaaaacccgcatgtcaaacccgactgggaaaacgtggagtttgcgctctttatgggcacctccccggcacagtccggcaatccgtttaaacgccaggcacgtcagttggcgagcgcccgactgcgtgagaattttcaatacgtcgtggtcgcccccgccctccccttatcaacggtgctcgccgatcctcgcggtcgctggcaaccggtcatgcccggcagtgattcggcgctggcaatggggatgatccgctggatcatggataatcaacgttataatgctgattatctggcgattcccggcgtacaggcgatgcagcaggccggcgagcaaagttggaccaacgccacgcacctggtcattgcggatgagctgccgacgcttgccggacaacacctgacgctgcgccatcttacgcccgatggcgaagagacccctgtcgtactgaataccgacggcgagttggtcgatgcgtccacttgccgacaggcacggcttttcgtgacgcagtacgttacgctcgccgacggccaacgggtcacggtgaagagcgggttgcaacgcctgaaagaggcggcagaaaagctctcgttggcgcaatacagcgaacagtgcggcgtgccggaagcgcaaattatcgcgctggcggaaacctttaccagtcacggacgtaaagctgcggtcatcagtcacggcggcatgatggccggcaatgggttttataacgcctggtcggtcatgatgcttaacgcgctgatcggcaacctcagcttgtccggcggcgtctttgtcggcggcggcaaattcaacggcgttagcgacggcccccgctacaacatgaacagttttgccggaaaagtgaaaccgtccgggttaagtattgcccgtagcaaaaccgcttatgaagcatcggaagaataccgcgacaaaattgccggtgggcaatccccttatccagccaaagcgccgtggtatccctttgtggcaggccagcttaccgaactgttgacctccgcgctcgaaggctatccttatccgcttaaagcctggatttccaatatgagcaacccgttttacggtgttcccggtctacgcgccgtggcggaagaaaaactaaaagaccctcgccgactgccgctctttatcgcgattgacgcctttatgaatgaaacgacggcgctggcggattacattgtgccggatacgcacaattttgagagctggggctttacggcgccctggggcggcgtagccagtaaagccactaccgcccgctggccggttgtcgcccccgccactcaccgcacggcggacgggcaacctgtctcaatggaagcattttgtattgcggtagcaaaacggctccatctgcccggcttcggcgaccgggcgataaccgatccgcagggcaatacttttccactgaaccgggcggaagacttctatctgcgcgtagccgctaatatcgcctttatgggcaagacgccggtcgcgctggcaaatcaggaagatatttcgcttaccggcgtcagccgcattctgccagcaattcagcacacgcttaaagctgatgaggtcggtcgcgtggcgtttatctactcgcgtggcggccggtttgcgcccgaggatagcggctatacggagcaacggttaggtaacgcgtggaaaaaacccttacagatctggaatgcagatgtcgccgcccaccgtcacgccatcaccggggagcgcttcagcggttgcccggtctggtatccggcgcgtttgtcagatggtcgtgcgattgacgaccagtttcccattgggcaatggccgctgaaactgatttcatttaaatcaaataccatgtccagctcaacagccgtcatcccgcgcttacaccatgtgaagccagcaaacctggtggcgctgaatccgcaagacggcgagcgttatggactgcaacatggcgatcgggtacggatcattacgccgggcggtcaggtcgtggcgcaaatcagtttgttaaatggcgtgatgccaggcgtcatcgccatcgaacacggatatggccaccgcgagatgggcgcaacgcagcactctctggatggcgtgcctatgccgtatgatccacaaatcagggcaggcataaatcttaacgatctgggctttgccgatccgacaagaaccattaccaacacctggctcgactgggtttctggcgcggcagtacgtcaggggctgccggcaaaaatcgagcgtata

SEQ ID NO: 34 - protein, 1020 aa, Salmonella enterica
MANLTRRQWLKVGLAVGGMVTFGLSYRDVAKRAIDGLLNGTSGKVTRDRIFGNALIPEAQAQTHWQQNPQQTIAMTQCFGCWTQCGIRARVNADGKVIRIAGNPYHPLSQEHPIDSSVPFSEAMEQLAGESGLDARSTACARGATLLESLYSPLRLLEPMKRVGKRGEGKWQRISFEQLIEEVVEGGDLFGEGHVDGLRAIHAPDTPIDAKHPSFGPKTNQLLVTNTSDEGRDAFLRRFALNSFGSKNFGAHGAYCGLAYRAGSGALMGDLDKNPHVKPDWENVEFALFMGTSPAQSGNPFKRQARQLASARLRENFQYVVVAPALPLSTVLADPRGRWQPVMPGSDSALAMGMIRWIMDNQRYNADYLAIPGVQAMQQAGEQSWTNATHLVIADELPTLAGQHLTLRHLTPDGEETPVVLNTDGELVDASTCRQARLFVTQYVTLADGQRVTVKSGLQRLKEAAEKLSLAQYSEQCGVPEAQIIALAETFTSHGRKAAVISHGGMMAGNGFYNAWSVMMLNALIGNLSLSGGVFVGGGKFNGVSDGPRYNMNSFAGKVKPSGLSIARSKTAYEASEEYRDKIAGGQSPYPAKAPWYPFVAGQLTELLTSALEGYPYPLKAWISNMSNPFYGVPGLRAVAEEKLKDPRRLPLFIAIDAFMNETTALADYIVPDTHNFESWGFTAPWGGVASKATTARWPVVAPATHRTADGQPVSMEAFCIAVAKRLHLPGFGDRAITDPQGNTFPLNRAEDFYLRVAANIAFMGKTPVALANQEDISLTGVSRILPAIQHTLKADEVGRVAFIYSRGGRFAPEDSGYTEQRLGNAWKKPLQIWNADVAAHRHAITGERFSGCPVWYPARLSDGRAIDDQFPIGQWPLKLISFKSNTMSSSTAVIPRLHHVKPANLVALNPQDGERYGLQHGDRVRIITPGGQVVAQISLLNGVMPGVIAIEHGYGHREMGATQHSLDGVPMPYDPQIRAGINLNDLGFADPTRTITNTWLDWVSGAAVRQGLPAKIERI

SEQ ID NO: 35 - DNA, 752 bp, Salmonella enterica
  source 1..752: mol_type = genomic DNA
atgtggacgggagtcaatatggacagcagtaaacggcaatttctccagcagcttggcgtcctgaccgctggcgcctcgctggttccgctggctgaagcgaaatttcctttttcgccggagcggcatgaaggctctccccgacaccgttacgccatgcttatcgatctgcggcgttgtatcggctgtcagtcctgtaccgtaagttgcactattgaaaaccaaacgccgcaaggcgcgtttcgtacgacggtgaaccaataccaggtccagcgtgaaggtagtcaggaagtcacgaatgtgctgttgccgcgtctgtgcaaccattgcgataaccccccctgtgtgccggtctgcccggtacaagccacctttcagcgggaagatggcattgtggtggtggataacaaacgctgcgtcggctgcgcctattgtgtccaggcgtgtccttacgacgcccgatttatcaatcatgaaacgcaaactgccgataaatgcacgttttgcgtccatcgtctggaagccggactgttacccgcttgcgtagagtcctgcgtcggcggcgcgcgtattattggcgatatcaaagatccccatagccgcatcgccaccatgcttcatcagcatcgcgacgctatcaaggtattaaagccggaaaacggcacgtcgccccatgttttctacctgggtctggacgacgcctttgtcaccccattaatgggccgtgcgcagcccgcgctttggcaggaggtctg

SEQ ID NO: 36 - protein, 250 aa, Salmonella enterica
MWTGVNMDSSKRQFLQQLGVLTAGASLVPLAEAKFPFSPERHEGSPRHRYAMLIDLRRCIGCQSCTVSCTIENQTPQGAFRTTVNQYQVQREGSQEVTNVLLPRLCNHCDNPPCVPVCPVQATFQREDGIVVVDNKRCVGCAYCVQACPYDARFINHETQTADKCTFCVHRLEAGLLPACVESCVGGARIIGDIKDPHSRIATMLHQHRDAIKVLKPENGTSPHVFYLGLDDAFVTPLMGRAQPALWQEV

SEQ ID NO: 37 - DNA, 1019 bp, Salmonella enterica
  source 1..1019: mol_type = genomic DNA
atgacgcattcactcatcattgaagaagtgctggctcacccgcaggacattagctggctgccgtgggcggtacaatatttcttttttattggcattgccgcctgcgccgcactgtttgcctgttatcttcactggcggaaaaaagacgccgcaacagaagaaaatcgggcattactgattgccattacctgtgcgattaccgcaccgctggcgctgacggcggatctgcaccagaccgcccgcgtctggcatttctatgcctggccgacgccctggtcgtggatgccctggggagcgttattcctgccgctgtttaccggatttctcgctctgtggttcctggcgcagcagattaaacgattattcaataaaagttacaacgtcactaaatggttggcgttagccagcgcgctttgcgcggtgggcctgttgatttataccggccgcgaagtctccgttgtgctggcgcgcccaatctggtttagctacgccttccccgtggcgatgtttcttagcgccttacaggcgttcttcgcgctgatgattgtcgccgcccgacgcgactcggtaaggctgccaaaaatattgtggggacaaatctggacgctggcggcgctggggctggttgtggccatgtgggttagcggcgatacgctttccggcacggcaatccgtcagtggattaccgtcgccctgtcagccaaatattacgctgtcggctgggtagcgctgtgggtatgcacactgctgttctgtagcctggcgctacgccatccgttatcacagctaagacgcgtcctgctggttctcagcgcgctggcgctatgttggctgatgcgctggacattgttgattcaggtacaaaccgtccccaagttcaacgcgcaatttaacccttactcgttaccaggcggaacggatggctggctggctattctcggcaccttcggcctgtggatagcgctactgattattattcgtgaaacgctgaacggactcaccaggagattacaacatgg

SEQ ID NO: 38 - protein, 340 aa, Salmonella enterica
MTHSLIIEEVLAHPQDISWLPWAVQYFFFIGIAACAALFACYLHWRKKDAATEENRALLIAITCAITAPLALTADLHQTARVWHFYAWPTPWSWMPWGALFLPLFTGFLALWFLAQQIKRLFNKSYNVTKWLALASALCAVGLLIYTGREVSVVLARPIWFSYAFPVAMFLSALQAFFALMIVAARHDSVRLPKILWGQIWTLAALGLVVAMWVSGDTLSGTAIRQWITVALSAKYYAVGWVALWVCTLLFCSLALRHPLSQLRRVLLVLSALALCWLMRWTLLIQVQTVPKFNAQFNPYSLPGGTDGWLAILGTFGLWIALLIIIRETLNGLTRRLQHG

SEQ ID NO: 39 - DNA, 639 bp, Salmonella enterica
  source 1..639: mol_type = genomic DNA
atgaaaatgggggcagggatggcgacaattcatctactggatgatgatacggcggtcactaacgcgtgcgcgtttttactggaaagtctgggatatgacgtaaaatgctggacgcagggggcggattttttggcgcaggccagtctgtatcaggccggggtcgtattactggatatgcgaatgccggtactggatgggcagggcgttcatgatgcgttgcgccagtgcggaagtaccctggcggttgtttttcttaccgggcatggcgatgtaccgatggccgtggagcagatgaaacgcggcgccgtcgattttctgcaaaaaccggtatcggtaaaaccgctacaggcggcgctggagcgtgcgctgacggtttcatcggcagcggtggcgcgtcgtgagattatactgtgttaccagcagttgacgccgaaagagcgtgagctggccagcctggtggcaaaaggatttatgaaccgtgaaattgcggaagcgatgaatatcgcggtgcgtaccgtagaggtgcaccgcgccagagtcatggaaaaaatgcaggccggtagcctggcggaactgattaggcgtttcgaaaaaatggcctcgccagagaccagaatacgaacaacgtatgagccatga

SEQ ID NO: 40 - protein, 212 aa, Salmonella enterica
MKMGAGMATIHLLDDDTAVTNACAFLLESLGYDVKCWTQGADFLAQASLYQAGVVLLDMRMPVLDGQGVHDALRQCGSTLAVVFLTGHGDVPMAVEQMKRGAVDFLQKPVSVKPLQAALERALTVSSAAVARREIILCYQQLTPKERELASLVAKGFMNREIAEAMNIAVRTVEVHRARVMEKMQAGSLAELIRRFEKMASPETRIRTTYEP

SEQ ID NO: 41 - DNA, 1779 bp, Salmonella enterica
  source 1..1779: mol_type = genomic DNA
gtgagaggtaaaaccgtaaggcgcctggcggtgttggcggcagtagggctactttgtcatggcgcgtgggcagggacgtggaatatcggtattttggccatgcgcggcgaggcgtctacgcgtagccactggcaaccgttggcaaagacattaagccaacagcttccaggcgaaacctttcacatccagccgctggatctgcatcaaatgcaggaggccgttaaccagggaaccgtgcagtttgtgataaccaacccggcgcaatttgtccaactgaacagccatgcgccgctgcgctggttagcttccctgcgctccacgcgcgatgggaaagcggtgagtaatgttattggcagcgtgattttgacccggcgcgatagcggcatcaccacggcgcatgatctcatcggtaagaccgtcggcgcgattgatgctcaggcgtttggcggctatttattaggctataaagcgctcagcgacgcgggcttacgcccggagcgcgattttcatctccgttttaccggatttcctggcgatgccttagtctatatgctgcgcgaaaaagcggtgcaggcggcaattgtgccagtgtgcctgttagaaaatatggatcaggaaggattgattaataaaaaggactttatcgcgctgctttcccgaccgacgcccctgccttgcttaaccagtacgccgttatatcctgactggtcgttcgcggcgctacctgcggtaagcgatgcgctggcggatcgcgtaacgcgagcgctattcaacgcgcccgccgccgcgtcatttcactggggcgcgcctgcgtccaccagtcaggtggaagccttgctgcgtgatgttcgtcagcaccctcagcagcgtcgactgtggctggatgtcaaaagttggttaatccagcaccagctaatggtcggcggcgtgattctggcgttcttgttgctcacgctcaattatatttgggtcatgctgctggtgcgtcgacgtggaaagcaactggaacgtaatagcgtagttcttcatcagcatgagcgggcgctggaaaccgcccggcaaatgagcgtgttgggtgaaatgacctccgggtttgcccatgagcttaatcagccgctttccgcgattcgacattatgcccaggggtgcctgattcgactgcgcgctgcagatgaacagcatcccttgctgccggcgctggagcagattgaccagcaggcgcaacgcggtgcggatactctgcgtaacctgcgtcactgggtcagccaggcgcagggcaacccggtgctaaccgaagcgtggaaggccatagccattcgcgaggcgattgatcatgtctggcaattgttgcgtatggcgcaacagtttccgacagtgactctgcataccgaggttagcgctgcgctgcgcgtaacgctgccgtcagtgctgctggaacaggtgctggcgaatatcattcttaatgcggctcaggcgggcgccacccatttatggatcgttgctgaacgcactgaaaacggcatcagtattgttttacaggataacgccgggggaatcgatgaggcgctattacgtcaggcgtttcagccgtttatgaccacccgtaaagaggggatgggcttagggctggcgatttgccagcggctggtgcggtatgggcggggcgatatcagcatcaggaaccagaccgcgccggacggtctgtcgggaacggtggttacgatacatttcttacatgaaaatgggggcagggatggcgacaattcatctactggatga

SEQ ID NO: 42 - protein, 592 aa, Salmonella enterica
MRGKTVRRLAVLAAVGLLCHGAWAGTWNIGILAMRGEASTRSHWQPLAKTLSQQLPGETFHIQPLDLHQMQEAVNQGTVQFVITNPAQFVQLNSHAPLRWLASLRSTRDGKAVSNVIGSVILTRRDSGITTAHDLIGKTVGAIDAQAFGGYLLGYKALSDAGLRPERDFHLRFTGFPGDALVYMLREKAVQAAIVPVCLLENMDQEGLINKKDFIALLSRPTPLPCLTSTPLYPDWSFAALPAVSDALADRVTRALFNAPAAASFHWGAPASTSQVEALLRDVRQHPQQRRLWLDVKSWLIQHQLMVGGVILAFLLLTLNYIWVMLLVRRRGKQLERNSVVLHQHERALETARQMSVLGEMTSGFAHELNQPLSAIRHYAQGCLIRLRAADEQHPLLPALEQIDQQAQRGADTLRNLRHWVSQAQGNPVLTEAWKAIAIREAIDHVWQLLRMAQQFPTVTLHTEVSAALRVTLPSVLLEQVLANIILNAAQAGATHLWIVAERTENGISIVLQDNAGGIDEALLRQAFQPFMTTRKEGMGLGLAICQRLVRYGRGDISIRNQTAPDGLSGTVVTIHFLHENGGRDGDNSSTG

SEQ ID NO: 43 - DNA, 5234 bp, synthetic construct
  misc_feature 1..5234: note = vector
  source 1..5234: mol_type = other DNA
aggcacacgaaaaacaagttaagggatgcagtttatcgggcagcgttgggtcctggccacgggtgcgcatgatcgtgctcctgtcgttgaggacccggctaggctggcggggttgccttactggttagcagaatgaatcaccgatacgcgagcgaacgtgaagcgactgctgctgcaaaacgtctgcgacctgagcaacaacatgaatggtcttcggtttccgtgtttcgtaaagtctggaaacgcggaagtcagcgccctgcaccattatgttccggatctgcatcgcaggatgctgctggctaccctgtggaacacctacatctgtattaacgaagcgctggcattgaccctgagtgatttttctctggtcccgccgcatccataccgccagttgtttaccctcacaacgttccagtaaccgggcatgttcatcatcagtaacccgtatcgtgagcatcctctctcgtttcatcggtatcattacccccatgaacagaaatcccccttacacggaggcatcagtgaccaaacaggaaaaaaccgcccttaacatggcccgctttatcagaagccagacattaacgcttctggagaaactcaacgagctggacgcggatgaacaggcagacatctgtgaatcgcttcacgaccacgctgatgagctttaccgcagctgcctcgcgcgtttcggtgatgacggtgaaaacctctgacacatgcagctcccggagacggtcacagcttgtctgtaagcggatgccgggagcagacaagcccgtcagggcgcgtcagcgggtgttggcgggtgtcggggcgcagccatgacccagtcacgtagcgatagcggagtgtatactggcttaactatgcggcatcagagcagattgtactgagagtgcaccatatgcggtgtgaaataccgcacagatgcgtaaggagaaaataccgcatcaggcgctcttccgcttcctcgctcactgactcgctgcgctcggtcgttcggctgcggcgagcggtatcagctcactcaaaggcggtaatacggttatccacagaatcaggggataacgcaggaaagaacatgtgagcaaaaggccagcaaaaggccaggaaccgtaaaaaggccgcgttgctggcgtttttccataggctccgcccccctgacgagcatcacaaaaatcgacgctcaagtcagaggtggcgaaacccgacaggactataaagataccaggcgtttccccctggaagctccctcgtgcgctctcctgttccgaccctgccgcttaccggatacctgtccgcctttctcccttcgggaagcgtggcgctttctcatagctcacgctgtaggtatctcagttcggtgtaggtcgttcgctccaagctgggctgtgtgcacgaaccccccgttcagcccgaccgctgcgccttatccggtaactatcgtcttgagtccaacccggtaagacacgacttatcgccactggcagcagtcccttaacttacttattaaataatttatagctattgaaaagagataagaattgttcaaagctaatattgtttaaatcgtcaattcctgcatgttttaaggaattgttaaattgattttttgtaaatattttcttgtattctttgttaacccatttcataacgaaataattatacttttgtttatctttgtgtgatattcttgatttttttctacttaatctgataagtgagctattcactttaggtttaggatgaaaatattctcttggaaccatacttaatatagaaatatcaacttctgccattaaaagtaatgccaatgagcgttttgtatttaataatcttttagcaaacccgtattccacgattaaataaatctcattagctatactatcaaaaacaattttgcgtattatatccgtacttatgttataaggtatattaccatatattttataggattggtttttaggaaatttaaactgcaatatatccttgtttaaaacttggaaattatcgtgatcaacaagtttattttctgtagttttgcataatttatggtctatttcaatggcagttacgaaattacacctctttactaattcaagggtaaaatggccttttcctgagccgatttcaaagatattatcatgttcatttaatcttatatttgtcattattttatctatattatgttttgaagtaataaagttttgactgtgttttatatttttctcgttcattataaccctctttaatttggttatatgaattttgcttattaacgattcattataaccacttattttttgtttggttgataatgaactgtgctgattacaaaaatactaaaaatgcccatattttttcctccttataaaattagtataattatagcacgagctctgataaatatgaacatgatgagtgatcgttaaatttatactgcaatcggatgcgattattgaataaaagatatgagagatttatctaatttcttttttcttgtaaaaaaagaaagttcttaaaggttttatagttttggtcgtagagcacacggtttaacgacttaattacgaagtaaataagtctagtgtgttagactttatgaaatctatatacgtttatatatatttattatccgattttttattaaaacgtctcaaaatcgtttctgagacgttttagcgtttatttcgtttagttatcggcataatcgttaaaacaggcgttatcgtagcgtaaaagcccttgagcgtagcgtggctttgcagcgaagatgttgtctgttagattatgaaagccgatgactgaatgaaataataagcgcagcgcccttctatttcggttggaggaggctcaagggagtatgagggaatgaaattccctcatgggtttgattttaaaaattgcttgcaattttgccgagcggtagcgctggaaaatttttgaaaaaaatttggaatttggaaaaaaatggggggaaaggaagcgaattttgcttccgtactacgaccccccattaagtgccgagtgccaatttttgtgccaaaaacgctctatcccaactggctcaagggtttaaggggtttttcaatcgccaacgaatcgccaacgttttcgccaacgttttttataaatctatatttaagtagctttattgttgtttttatgattacaaagtgatacactaactttataaaattatttgattggagttttttaaatggtgatttcagaatcgaaaaaaagagttatgatttctctgacaaaagagcaagataaaaaattaacagatatggcgaaacaaaaaggtttttcaaaatctgcggttgcggcgttagctatagaagaatatgcaagaaaggaatcagaacaaaaaaaataagcgaaagctcgcgtttttagaaggatacgagttttcgctacttgtttttgataaggtaattatatcatggctattaaaaatactaaagctagaaattttggatttttattatatcctgactcaattcctaatgattggaaagaaaaattagagagtttgggcgtatctatggctgtcagtcctttacacgatatggacgaaaaaaaagataaagatacatggaataatagtaatattatacaaaatggaaagcactataaaaaaccacactatcacgttatatatattgcacgaaatcctgtaacaatagaaagcgttaggaacaagattaagcgaaaattggggaatagttcagttgctcatgttgagatacttgattatatcaaaggttcatatgaatatttgactcatgaatcaaaggacgctattgctaagaataaacatatatacgacaaaaaagatattttgaacattaatgattttgatattgaccgctatataacacttgatgaaagccaaaaaagagaattgaagaatttacttttagatatagtggatgactataatttggtaaatacaaaagatttaatggcttttattcgccttaggggagcggagtttggaattttaaatacaaagatattgtttcaacaaagaatgatgtactctagcgcctttagattatggtttgagggcaattatcagtgtggatatagagcaagttatgcaaaggttcttgatgctgaaacgggggaaataaaatgacaaacaaagaaaaagagttatttgctgaaaatgaggaattaaaaaaagaaattaaggacttaaaagagcgtattgaaagatacagagaaatggaagttgaattaagtacaacaatagatttattgagaggagggattattgaataaataaaagccccctgacgaaagtcgaagggggtttttattttggtttgatgttgcgattaatagcaatacaattgcaataaacaaaatgatcttccttcaggttatgaccatctgtgccagttcgtaatgtctggtcaactttccgactctgagaaacttctggaatcgctagagaatttctggaatgggattcaggagtggacagaacgacacggatatatagtggatgtgtcaaaacgcataccattttgaacgatgacctctaataattgttaatcatgttggttacgtatttattaacttctcctagtattagtaattatcatggctgtcatggcgcattaacggaataaagggtgtgcttaaatcgggccattttgcgtaataagaaaaaggattaattatgagcgaattgaattaataataaggtaatagatttacattagaaaatgaaaggggattttatgcgtgagaatgttacagtctatccctggcgaaagggggatgtgctgcaaggcgattaagttgggtaacgccagggttttcccagtcacgacgttgtaaaacgacggccagtgagcgcgcgtaatacgactcactatagggcgaattgggtaccgggccccccctcgaggtcgacggtatcgataagcttgatatcgaattcctgcagcccgggggatccactagttctagagcggccgccaccgcggtggagctccagcttttgttccctttagtgagggttaattgcgcgcttggcgtaatcatggtcatagctgtttcctgtgtgaaattgttatccgctcacaattccacacaacatacgagccggaagcataaagtgtaaagcctggggtgcctaatgagtgagctaactcacattaattgcgttgcgctcactgcccgctttccagtcgggaaacctgtcgtgccag

SEQ ID NO: 44 - DNA, 5234 bp, synthetic construct; identical to SEQ ID NO: 43
  misc_feature 1..5234: note = vector
  source 1..5234: mol_type = other DNA

SEQ ID NO: 45 - DNA, 4500 bp, synthetic construct
  misc_feature 1..4500: note = vector
  source 1..4500: mol_type = other DNA
ttccccttctctgaaaatcaacgggcaggtcactgacttgcccgtttttttatcccttctccacaccgttgagctcgaattctcatgtttgacagcttatcactgatcagtgaattaatggcgatgacgcatcctcacgataatatccgggtaggcgcaatcactttcgtctctactccgttacaaagcgaggctgggtatttcccggcctttctgttatccgaaatccactgaaagcacagcggctggctgaggagataaataataaacgaggggctgtatgcacaaagcatcttctgttgagttaagaacgagtatcgagatggcacatagccttgctcaaattggaatcaggtttgtgccaataccagtagaaacagacgaagaagctagaggtgaatcacgacaaagcgtatcaaaaacgtatggagtagggctctaaactctgtataaaaagtttccagctagctgataacgggaaagaaacagagaagggcacaaatattgtgtactttaatgtgccctttaatttattgattggtggttgaattgtccgtaactttttgatttaagtgcaaatttctaataaattagaacactttcttaaattgtcatttggcatattacgaacaattccgcgtaaaaacgttctgttacgctaaacccttatccagcaggctttcaaggatgtaaaccataacactctgcgaactagtgttacattgcgtgtagctttgagtgggcaactttgtgtacacttttgtgtacccaaaaacaaaaatgtgtacccattcaatgatcaccgacacaaagctcaggaaggcgctcggcaagaaaagagatgatatcgagattatttctgattcgcacgagctttctagacgctcaagttagtataaaaaagctgaacgagaaacgtaaaatgatataaatatcaatatattaaattagattttgcataaaaaacagactacataatactgtaaaacacaacatatgcagtcactatgaatcaactacttagatggtattagtgacctgtaacagactgcgggcccaggttatgctgcttttaagacccactttcacatttaagttgtttttctaatccgcatatgatcaattcaaggccgaataagaaggctggctctgcaccttggtgatcaaataattcgatagcttgtcgtaataatggcggcatactatcagtagtaggtgtttccctttcttctttagcgacttgatgctcttgatcttccaatacgcaacctaaagtaaaatgccccacagcgctgagtgcatataatgcattctctagtgaaaaaccttgttggcataaaaaggctaattgattttcgagagtttcatactgtttttctgtaggccgtgtacctaaatgtacttttgctccatcgcgatgacttagtaaagcacatctaaaacttttagcgttattacgtaaaaaatcttgccagctttccccttctaaagggcaaaagtgagtatggtgcctatctaacatctcaatggctaaggcgtcgagcaaagcccgcttattttttacatgccaatacaatgtaggctgctctacacctagcttctgggcgagtttacgggttgttaaaccttcgattccgacctcattaagcagctctaatgcgctgttaatcactttacttttatctaatctagacatcattaattcctaatttttgttgacactctatcattgatagagttattttaccactccctatcagtgatagagaaaagtgaaatgaatagttcgacaaagatcgcattggtaattacgttactcgatgccatggggattggccttatcatgccagtcttgccaacgttattacgtgaatttattgcttcggaagatatcgctaaccactttggcgtattgcttgcactttatgcgttaatgcaggttatctttgctccttggcttggaaaaatgtctgaccgatttggtcggcgcccagtgctgttgttgtcattaataggcgcatcgctggattacttattgctggctttttcaagtgcgctttggatgctgtatttaggccgtttgctttcagggatcacaggagctactggggctgtcgcggcatcggtcattgccgataccacctcagcttctcaacgcgtgaagtggttcggttggttaggggcaagttttgggcttggtttaatagcggggcctattattggtggttttgcaggagagatttcaccgcatagtcccttttttatcgctgcgttgctaaatattgtcactttccttgtggttatgttttggttccgtgaaaccaaaaatacacgtgataatacagataccgaagtaggggttgagacgcaatcgaattcggtatacatcactttatttaaaacgatgcccattttgttgattatttatttttcagcgcaattgataggccaaattcccgcaacggtgtgggtgctatttaccgaaaatcgttttggatggaatagcatgatggttggcttttcattagcgggtcttggtcttttacactcagtattccaagcctttgtggcaggaagaatagccactaaatggggcgaaaaaacggcagtactgctcgaatttattgcagatagtagtgcatttgcctttttagcgtttatatctgaaggttggttagatttccctgttttaattttattggctggtggtgggatcgctttacctgcattacagggagtgatgtctatccaaacaaagagtcatgagcaaggtgctttacagggattattggtgagccttaccaatgcaaccggtgttattggcccattactgtttactgttatttataatcattcactaccaatttgggatggctggatttggattattggtttagcgttttactgtattattatcctgctatcgatgaccttcatgttaacccctcaagctcaggggagtaaacaggagacaagtgcttagttatttcgtcaccaaatgatgttattccgcgaaatataatgaccctcttgataacccaagagggcattttttacgagacgtcctaattcccatgtcagccgttaagtgttcctgtgtcactgaaaattgctttgagaggctctaagggcttctcagtgcgttacatccctggcttgttgtccacaaccgttaaaccttaaaagctttaaaagccttatatattcttttttttcttataaaacttaaaaccttagaggctatttaagttgctgatttatattaattttattgttcaaacatgagagcttagtacgtgaaacatgagagcttagtacgttagccatgagagcttagtacgttagccatgagggtttagttcgttaaacatgagagcttagtacgttaaacatgagagcttagtacgtgaaacatgagagcttagtacgtactatcaacaggttgaactgctgatcttcagatcctctacgccggacgcatcgtggccggatcttgcggccgcaaaaattaaaaatgaagttttggaggcctcatttggtgacgaaataactaagcacttgtctcctgtttactcccctgagcttgaggggtcaacatgaaggtcattgatagcaggataataatacagtaaaacgctaaaccaataatccaaatccagccatcccaaattggtagtgaatgattataaataacagtaaacagtaatgggccaataacaccggttgcattggtaaggctcaccaataatccctgtaaagcaccttgctcatgactctttgtttggatagacatcactccctgtaatgcaggtaaagcgatcccaccaccagccaataaaattaaaacagggaaatctaaccaaccttcagatataaacgctaaaaaggcaaatgcactactatctgcaataaattcgagcagtactgccgttttttcgccccatttagtggctattcttcctgccacaaaggcttggaatactgagtgtaaaagaccaagacccgctaatgaaaagccaaccatcatgctattccatccaaaacgattttcggtaaatagcacccacaccgttgcgggaatttggcctatcaattcgaaatcaaataatgattttattttgactgatagtgacctgttcgttgcaacaaattgataagcaatgcttttttataatgccaacttagtataaaaaagcaggcttcagagcgatggcccccgatggtagtgtggggtctccccatgcgagagtagggaactgccaggcatcaaataaaacgaaaggctcagtcgaaagactgggcctttcgttttatctgttgtttgtcggtgaacgctctcctgagtaggacaaatccgccgggagcggatttgaacgttgcgaagcaacggcccggagggtggcgggcaggacgcccgccataaactgccaggcatcaaattaagcagaaggccatcctgacggatggcctttttgcgtggccagtgccaagcttgcatgc

SEQ ID NO: 46 - DNA, 10255 bp, synthetic construct
  misc_feature 1..10255: note = vector
  source 1..10255: mol_type = other DNA
ctgcaggtcgactctagaggatccgttatatacgctcgatttttgccggcagcccctgacgtactgccgcgccagaaacccagtcgagccaggtgttggtaatggttcttgtcggatcggcaaagcccagatcgttaagatttatgcctgccctgatttgtggatcatacggcataggcacgccatccagagagtgctgcgttgcgcccatctcgcggtggccatatccgtgttcgatggcgatgacgcctggcatcacgccatttaacaaactgatttgcgccacgacctgaccgcccggcgtaatgatccgtacccgatcgccatgttgcagtccataacgctcgccgtcttgcggattcagcgccaccaggtttgctggcttcacatggtgtaagcgcgggatgacggctgttgagctggacatggtatttgatttaaatgaaatcagtttcagcggccattgcccaatgggaaactggtcgtcaatcgcacgaccatctgacaaacgcgccggataccagaccgggcaaccgctgaagcgctccccggtgatggcgtgacggtgggcggcgacatctgcattccagatctgtaagggttttttccacgcgttacctaaccgttgctccgtatagccgctatcctcgggcgcaaaccggccgccacgcgagtagataaacgccacgcgaccgacctcatcagctttaagcgtgtgctgaattgctggcagaatgcggctgacgccggtaagcgaaatatcttcctgatttgccagcgcgaccggcgtcttgcccataaaggcgatattagcggctacgcgcagatagaagtcttccgcccggttcagtggaaaagtattgccctgcggatcggttatcgcccggtcgccgaagccgggcagatggagccgttttgctaccgcaatacaaaatgcttccattgagacaggttgcccgtccgccgtgcggtgagtggcgggggcgacaaccggccagcgggcggtagtggctttactggctacgccgccccagggcgccgtaaagccccagctctcaaaattgtgcgtatccggcacaatgtaatccgccagcgccgtcgtttcattcataaaggcgtcaatcgcgataaagagcggcagtcggcgagggtcttttagtttttcttccgccacggcgcgtagaccgggaacaccgtaaaacgggttgctcatattggaaatccaggctttaagcggataaggatagccttcgagcgcggaggtcaacagttcggtaagctggcctgccacaaagggataccacggcgctttggctggataaggggattgcccaccggcaattttgtcgcggtattcttccgatgcttcataagcggttttgctacgggcaatacttaacccggacggtttcacttttccggcaaaactgttcatgttgtagcgggggccgtcgctaacgccgttgaatttgccgccgccgacaaagacgccgccggacaagctgaggttgccgatcagcgcgttaagcatcatgaccgaccaggcgttataaaacccattgccggccatcatgccgccgtgactgatgaccgcagctttacgtccgtgactggtaaaggtttccgccagcgcgataatttgcgcttccggcacgccgcactgttcgctgtattgcgccaacgagagcttttctgccgcctctttcaggcgttgcaacccgctcttcaccgtgacccgttggccgtcggcgagcgtaacgtactgcgtcacgaaaagccgtgcctgtcggcaagtggacgcatcgaccaactcgccgtcggtattcagtacgacaggggtctcttcgccatcgggcgtaagatggcgcagcgtcaggtgttgtccggcaagcgtcggcagctcatccgcaatgaccaggtgcgtggcgttggtccaactttgctcgccggcctgctgcatcgcctgtacgccgggaatcgccagataatcagcattataacgttgattatccatgatccagcggatcatccccattgccagcgccgaatcactgccgggcatgaccggttgccagcgaccgcgaggatcggcgagcaccgttgataaggggagggcgggggcgaccacgacgtattgaaaattctcacgcagtcgggcgctcgccaactgacgtgcctggcgtttaaacggattgccggactgtgccggggaggtgcccataaagagcgcaaactccacgttttcccagtcgggtttgacatgcgggtttttatccagatcgcccatcaatgccccggagccggcccggtaagccagtccacagtaggcgccatgcgcgccgaaattcttgctgccgaagctatttagcgcaaaacgacgcagaaacgcatcgcggccttcgtcgctggtattcgtgaccagtaactgattggttttgggcccgaaactggggtgctttgcgtcaattggcgtatccggcgcatgaatagcgcgcagtccgtccacatgaccttcgccaaacagatcgccgccttccacgacttcttcaataagttgctcaaagctgatgcgctgccatttcccttcgccgcgtttacccacgcgtttcatcggttcaagcagtcgtagcggactgtacaggctttccagcagcgtggcgccgcgcgcgcaggcggttgagcgggcgtcaagaccgctttctcccgccagttgctccatggcttcgctaaaagggacggacgagtcaatcgggtgttcctgcgacaaggggtgatagggattgccggcgatgcgtatcactttgccatcggcattaacccgggcgcggataccgcactgtgtccaacagccgaagcattgcgtcatggcgatggtttgttgtggattttgctgccagtgtgtttgcgcctgcgcctccggaattaacgcattgccaaagatgcggtcgcgcgttaccttgccggacgtcccgtttaacaggccatcaattgcgcgtttcgccacatcacggtagctcagaccaaaagtgaccatcccaccgacggcgagaccgacttttagccactgacgacgggttaaattagccatgttgtaatctcctggtgagtccgttcagcgtttcacgaataataatcagtagcgctatccacaggccgaaggtgccgagaatagccagccagccatccgttccgcctggtaacgagtaagggttaaattgcgcgttgaacttggggacggtttgtacctgaatcaacaatgtccagcgcatcagccaacatagcgccagcgcgctgagaaccagcaggacgcgtcttagctgtgataacggatggcgtagcgccaggctacagaacagcagtgtgcatacccacagcgctacccagccgacagcgtaatatttggctgacagggcgacggtaatccactgacggattgccgtgccggaaagcgtatcgccgctaacccacatggccacaaccagccccagcgccgccagcgtccagatttgtccccacaatatttttggcagccttaccgagtcgcgtcgggcggcgacaatcatcagcgcgaagaacgcctgtaaggcgctaagaaacatcgccacggggaaggcgtagctaaaccagattgggcgcgccagcacaacggagacttcgcggccggtataaatcaacaggcccaccgcgcaaagcgcgctggctaacgccaaccatttagtgacgttgtaacttttattgaataatcgtttaatctgctgcgccaggaaccacagagcgagaaatccggtaaacagcggcaggaataacgctccccagggcatccacgaccagggcgtcggccaggcatagaaatgccagacgcgggcggtctggtgcagatccgccgtcagcgccagcggtgcggtaatcgcacaggtaatggcaatcagtaatgcccgattttcttctgttgcggcgtcttttttccgccagtgaagataacaggcaaacagtgcggcgcaggcggcaatgccaataaaaaagaaatattgtaccgcccacggcagccagctaatgtcctgcgggtgagccagcacttcttcaatgatgagtgaatgcgtcattcagacctcctgccaaagcgcgggctgcgcacggcccattaatggggtgacaaaggcgtcgtccagacccaggtagaaaacatggggcgacgtgccgttttccggctttaataccttgatagcgtcgcgatgctgatgaagcatggtggcgatgcggctatggggatctttgatatcgccaataatacgcgcgccgccgacgcaggactctacgcaagcgggtaacagtccggcttccagacgatggacgcaaaacgtgcatttatcggcagtttgcgtttcatgattgataaatcgggcgtcgtaaggacacgcctggacacaataggcgcagccgacgcagcgtttgttatccaccaccacaatgccatcttcccgctgaaaggtggcttgtaccgggcagaccggcacacagggggggttatcgcaatggttgcacagacgcggcaacagcacattcgtgacttcctgactaccttcacgctggacctggtattggttcaccgtcgtacgaaacgcgccttgcggcgtttggttttcaatagtgcaacttacggtacaggactgacagccgatacaacgccgcagatcgataagcatggcgtaacggtgtcggggagagccttcatgccgctccggcgaaaaaggaaatttcgcttcagccagcggaaccagcgaggcgccagcggtcaggacgccaagctgctggagaaattgccgtttactgctgtccatattgactcccgtccacattgccaacaatgaaacatttgtcacgatgttggttcatgtgtaatgaataaaaaatgtcgatgatttacagtgtaaaaatcgaggcggggtgcgctctattgtggttaaccacatacccggcttgttgttgatctaaaacaacataattgacagggatattggggtgagaggtaaaaccgtaaggcgcctggcggtgttggcggcagtagggctactttgtcatggcgcgtgggcagggacgtggaatatcggtattttggccatgcgcggcgaggcgtctacgcgtagccactggcaaccgttggcaaagacattaagccaacagcttccaggcgaaacctttcacatccagccgctggatctgcatcaaatgcaggaggccgttaaccagggaaccgtgcagtttgtgataaccaacccggcgcaatttgtccaactgaacagccatgcgccgctgcgctggttagcttccctgcgctccacgcgcgatgggaaagcggtgagtaatgttattggcagcgtgattttgacccggcgcgatagcggcatcaccacggcgcatgatctcatcggtaagaccgtcggcgcgattgatgctcaggcgtttggcggctatttattaggctataaagcgctcagcgacgcgggcttacgcccggagcgcgattttcatctccgttttaccggatttcctggcgatgccttagtctatatgctgcgcgaaaaagcggtgcaggcggcaattgtgccagtgtgcctgttagaaaatatggatcaggaaggattgattaataaaaaggactttatcgcgctgctttcccgaccgacgcccctgccttgcttaaccagtacgccgttatatcctgactggtcgttcgcggcgctacctgcggtaagcgatgcgctggcggatcgcgtaacgcgagcgctattcaacgcgcccgccgccgcgtcatttcactggggcgcgcctgcgtccaccagtcaggtggaagccttgctgcgtgatgttcgtcagcaccctcagcagcgtcgactgtggctggatgtcaaaagttggttaatccagcaccagctaatggtcggcggcgtgattctggcgttcttgttgctcacgctcaattatatttgggtcatgctgctggtgcgtcgacgtggaaagcaactggaacgtaatagcgtagttcttcatcagcatgagcgggcgctggaaaccgcccggcaaatgagcgtgttgggtgaaatgacctccgggtttgcccatgagcttaatcagccgctttccgcgattcgacattatgcccaggggtgcctgattcgactgcgcgctgcagatgaacagcatcccttgctgccggcgctggagcagattgaccagcaggcgcaacgcggtgcggatactctgcgtaacctgcgtcactgggtcagccaggcgcagggcaacccggtgctaaccgaagcgtggaaggccatagccattcgcgaggcgattgatcatgtctggcaattgttgcgtatggcgcaacagtttccgacagtgactctgcataccgaggttagcgctgcgctgcgcgtaacgctgccgtcagtgctgctggaacaggtgctggcgaatatcattcttaatgcggctcaggcgggcgccacccatttatggatcgttgctgaacgcactgaaaacggcatcagtattgttttacaggataacgccgggggaatcgatgaggcgctattacgtcaggcgtttcagccgtttatgaccacccgtaaagaggggatgggcttagggctggcgatttgccagcggctggtgcggtatgggcggggcgatatcagcatcaggaaccagaccgcgccggacggtctgtcgggaacggtggttacgatacatttcttacatgaaaatgggggcagggatggcgacaattcatctactggatgatgatacggcggtcactaacgcgtgcgcgtttttactggaaagtctgggatatgacgtaaaatgctggacgcagggggcggattttttggcgcaggccagtctgtatcaggccggggtcgtattactggatatgcgaatgccggtactggatgggcagggcgttcatgatgcgttgcgccagtgcggaagtaccctggcggttgtttttcttaccgggcatggcgatgtaccgatggccgtggagcagatgaaacgcggcgccgtcgattttctgcaaaaaccggtatcggtaaaaccgctacaggcggcgctggagcgtgcgctgacggtttcatcggcagcggtggcgcgtcgtgagattatactgtgttaccagcagttgacgccgaaagagcgtgagctggccagcctggtggcaaaaggatttatgaaccgtgaaattgcggaagcgatgaatatcgcggtgcgtaccgtagaggtgcaccgcgccagagtcatggaaaaaatgcaggccggtagcctggcggaactgattaggcgtttcgaaaaaatggcctcgccagagaccagaatacgaacaacgtatgagccatgaataagagctcgaattctcatgtttgacagcttatcactgatcagtgaattaatggcgatgacgcatcctcacgataatatccgggtaggcgcaatcactttcgtctctactccgttacaaagcgaggctgggtatttcccggcctttctgttatccgaaatccactgaaagcacagcggctggctgaggagataaataataaacgaggggctgtatgcacaaagcatcttctgttgagttaagaacgagtatcgagatggcacatagccttgctcaaattggaatcaggtttgtgccaataccagtagaaacagacgaagaagctagaggtgaatcacgacaaagcgtatcaaaaacgtatggagtagggctctaaactctgtataaaaagtttccagctagctgataacgggaaagaaacagagaagggcacaaatattgtgtactttaatgtgccctttaatttattgattggtggttgaattgtccgtaactttttgatttaagtgcaaatttctaataaattagaacactttcttaaattgtcatttggcatattacgaacaattccgcgtaaaaacgttctgttacgctaaacccttatccagcaggctttcaaggatgtaaaccataacactctgcgaactagtgttacattgcgtgtagctttgagtgggcaactttgtgtacacttttgtgtacccaaaaacaaaaatgtgtacccattcaatgatcaccgacacaaagctcaggaaggcgctcggcaagaaaagagatgatatcgagattatttctgattcgcacgggcccatggctaattcccatgtcagccgttaagtgttcctgtgtcactgaaaattgctttgagaggctctaagggcttctcagtgcgttacatccctggcttgttgtccacaaccgttaaaccttaaaagctttaaaagccttatatattcttttttttcttataaaacttaaaaccttagaggctatttaagttgctgatttatattaattttattgttcaaacatgagagcttagtacgtgaaacatgagagcttagtacgttagccatgagagcttagtacgttagccatgagggtttagttcgttaaacatgagagcttagtacgttaaacatgagagcttagtacgtgaaacatgagagcttagtacgtactatcaacaggttgaactgctgatcttcagatcctctacgccggacgcatcgtggccggatcttgcggccgcaaaaattaaaaatgaagttttggaggcctcatttggtgacgaaataactaagcacttgtctcctgtttactcccctgagcttgaggggtcaacatgaaggtcattgatagcaggataataatacagtaaaacgctaaaccaataatccaaatccagccatcccaaattggtagtgaatgattataaataacagtaaacagtaatgggccaataacaccggttgcattggtaaggctcaccaataatccctgtaaagcaccttgctcatgactctttgtttggatagacatcactccctgtaatgcaggtaaagcgatcccaccaccagccaataaaattaaaacagggaaatctaaccaaccttcagatataaacgctaaaaaggcaaatgcactactatctgcaataaattcgagcagtactgccgttttttcgccccatttagtggctattcttcctgccacaaaggcttggaatactgagtgtaaaagaccaagacccgctaatgaaaagccaaccatcatgctattccatccaaaacgattttcggtaaatagcacccacaccgttgcgggaatttggcctatcaattgcgctgaaaaataaataatcaacaaaatgggcatcgttttaaataaagtgatgtacaccgaatttgattgcgtctcaacccctacttcggtatctgtattatcacgtgtatttttggtttcacggaaccaaaacataaccacaaggaaagtgacaatatttagcaacgcagcgataaaaaagggactatgcggtgaaatctctcctgcaaaaccaccaataataggccccgctattaaaccaagcccaaaacttgcccctaaccaaccgaaccacttcacgcgttgagaagctgaggtggtatcggcaatgaccgatgccgcgacagccccagtagctcctgtgatccctgaaagcaaacggcctaaatacagcatccaaagcgcacttgaaaaagccagcaataagtaatccagcgatgcgcctattaatgacaacaacagcactgggcgccgaccaaatcggtcagacatttttccaagccaaggagcaaagataacctgcattaacgcataaagtgcaagcaatacgccaaagtggttagcgatatcttccgaagcaataaattcacgtaataacgttggcaagactggcatgataaggccaatccccatggcatcgagtaacgtaattaccaatgcgatctttgtcgaactattcatttcacttttctctatcactgatagggagtgggaaaataactctatcaatgatagggtgtcaaatcgatggcccccgatggtagtgtggggtctccccatgcgagagtagggaactgccaggcatcaaataaaacgaaaggctcagtcgaaagactgggcctttcgttttatctgttgtttgtcggtgaacgctctcctgagtaggacaaatccgccgggagcggatttgaacgttgcgaagcaacggcccggagggtggcgggcaggacgcccgccataaactgccaggcatcaaattaagcagaaggccatcctgacggatggcctttttgcgtggccagtgccaagcttgcatgc

SEQ ID NO: 47 - DNA, 10465 bp, synthetic construct
  misc_feature 1..10465: note = vector
  source 1..10465: mol_type = other DNA
gacctataaggaaaggccaaacaagaacacggttgcaaaaaccgtgcccttaaatattgaatttctattcagaacactttcttaaattgtcatttggcatattacgaacaattccgcgtaaaaacgttctgttacgctaaacccttatccagcaggctttcaaggatgtaaaccataacactctgcgaactagtgttacattgcgtgtagctttgagtgggcaactttgtgtacacttttgtgtacccaaaaacaaaaatgtgtacccattcaatgatcaccgacacaaagctcaggaaggcgctcggcaagaaaagagatgatatcgagattatttctgattcgcacgggcccatggctaattcccatgtcagccgttaagtgttcctgtgtcactgaaaattgctttgagaggctctaagggcttctcagtgcgttacatccctggcttgttgtccacaaccgttaaaccttaaaagctttaaaagccttatatattcttttttttcttataaaacttaaaaccttagaggctatttaagttgctgatttatattaattttattgttcaaacatgagagcttagtacgtgaaacatgagagcttagtacgttagccatgagagcttagtacgttagccatgagggtttagttcgttaaacatgagagcttagtacgttaaacatgagagcttagtacgtgaaacatgagagcttagtacgtactatcaacaggttgaactgctgatcttcagatcctctacgccggacgcatcgtggccggatcttgcggccgcaaaaattaaaaatgaagttttggaggcctcatttggtgacgaaataactaagcacttgtctcctgtttactcccctgagcttgaggggtcaacatgaaggtcattgatagcaggataataatacagtaaaacgctaaaccaataatccaaatccagccatcccaaattggtagtgaatgattataaataacagtaaacagtaatgggccaataacaccggttgcattggtaaggctcaccaataatccctgtaaagcaccttgctcatgactctttgtttggatagacatcactccctgtaatgcaggtaaagcgatcccaccaccagccaataaaattaaaacagggaaatctaaccaaccttcagatataaacgctaaaaaggcaaatgcactactatctgcaataaattcgagcagtactgccgttttttcgccccatttagtggctattcttcctgccacaaaggcttggaatactgagtgtaaaagaccaagacccgctaatgaaaagccaaccatcatgctattccatccaaaacgattttcggtaaatagcacccacaccgttgcgggaatttggcctatcaattgcgctgaaaaataaataatcaacaaaatgggcatcgttttaaataaagtgatgtacaccgaatttgattgcgtctcaacccctacttcggtatctgtattatcacgtgtatttttggtttcacggaaccaaaacataaccacaaggaaagtgacaatatttagcaacgcagcgataaaaaagggactatgcggtgaaatctctcctgcaaaaccaccaataataggccccgctattaaaccaagcccaaaacttgcccctaaccaaccgaaccacttcacgcgttgagaagctgaggtggtatcggcaatgaccgatgccgcgacagccccagtagctcctgtgatccctgaaagcaaacggcctaaatacagcatccaaagcgcacttgaaaaagccagcaataagtaatccagcgatgcgcctattaatgacaacaacagcactgggcgccgaccaaatcggtcagacatttttccaagccaaggagcaaagataacctgcattaacgcataaagtgcaagcaatacgccaaagtggttagcgatatcttccgaagcaataaattcacgtaataacgttggcaagactggcatgataaggccaatccccatggcatcgagtaacgtaattaccaatgcgatctttgtcgaactattcatttcacttttctctatcactgatagggagtgggaaaataactctatcaatgatagggtgtcaaatcgatggcccccgatggtagtgtggggtctccccatgcgagagtagggaactgccaggcatcaaataaaacgaaaggctcagtcgaaagactgggcctttcgttttatctgttgtttgtcggtgaacgctctcctgagtaggacaaatccgccgggagcggatttgaacgttgcgaagcaacggcccggagggtggcgggcaggacgcccgccataaactgccaggcatcaaattaagcagaaggccatcctgacggatggcctttttgcgtggccagtgccaagcttgcatgcctgcaggtcgactctagaggatccgttatatacgctcgatttttgccggcagcccctgacgtactgccgcgccagaaacccagtcgagccaggtgttggtaatggttcttgtcggatcggcaaagcccagatcgttaagatttatgcctgccctgatttgtggatcatacggcataggcacgccatccagagagtgctgcgttgcgcccatctcgcggtggccatatccgtgttcgatggcgatgacgcctggcatcacgccatttaacaaactgatttgcgccacgacctgaccgcccggcgtaatgatccgtacccgatcgccatgttgcagtccataacgctcgccgtcttgcggattcagcgccaccaggtttgctggcttcacatggtgtaagcgcgggatgacggctgttgagctggacatggtatttgatttaaatgaaatcagtttcagcggccattgcccaatgggaaactggtcgtcaatcgcacgaccatctgacaaacgcgccggataccagaccgggcaaccgctgaagcgctccccggtgatggcgtgacggtgggcggcgacatctgcattccagatctgtaagggttttttccacgcgttacctaaccgttgctccgtatagccgctatcctcgggcgcaaaccggccgccacgcgagtagataaacgccacgcgaccgacctcatcagctttaagcgtgtgctgaattgctggcagaatgcggctgacgccggtaagcgaaatatcttcctgatttgccagcgcgaccggcgtcttgcccataaaggcgatattagcggctacgcgcagatagaagtcttccgcccggttcagtggaaaagtattgccctgcggatcggttatcgcccggtcgccgaagccgggcagatggagccgttttgctaccgcaatacaaaatgcttccattgagacaggttgcccgtccgccgtgcggtgagtggcgggggcgacaaccggccagcgggcggtagtggctttactggctacgccgccccagggcgccgtaaagccccagctctcaaaattgtgcgtatccggcacaatgtaatccgccagcgccgtcgtttcattcataaaggcgtcaatcgcgataaagagcggcagtcggcgagggtcttttagtttttcttccgccacggcgcgtagaccgggaacaccgtaaaacgggttgctcatattggaaatccaggctttaagcggataaggatagccttcgagcgcggaggtcaacagttcggtaagctggcctgccacaaagggataccacggcgctttggctggataaggggattgcccaccggcaattttgtcgcggtattcttccgatgcttcataagcggttttgctacgggcaatacttaacccggacggtttcacttttccggcaaaactgttcatgttgtagcgggggccgtcgctaacgccgttgaatttgccgccgccgacaaagacgccgccggacaagctgaggttgccgatcagcgcgttaagcatcatgaccgaccaggcgttataaaacccattgccggccatcatgccgccgtgactgatgaccgcagctttacgtccgtgactggtaaaggtttccgccagcgcgataatttgcgcttccggcacgccgcactgttcgctgtattgcgccaacgagagcttttctgccgcctctttcaggcgttgcaacccgctcttcaccgtgacccgttggccgtcggcgagcgtaacgtactgcgtcacgaaaagccgtgcctgtcggcaagtggacgcatcgaccaactcgccgtcggtattcagtacgacaggggtctcttcgccatcgggcgtaagatggcgcagcgtcaggtgttgtccggcaagcgtcggcagctcatccgcaatgaccaggtgcgtggcgttggtccaactttgctcgccggcctgctgcatcgcctgtacgccgggaatcgccagataatcagcattataacgttgattatccatgatccagcggatcatccccattgccagcgccgaatcactgccgggcatgaccggttgccagcgaccgcgaggatcggcgagcaccgttgataaggggagggcgggggcgaccacgacgtattgaaaattctcacgcagtcgggcgctcgccaactgacgtgcctggcgtttaaacggattgccggactgtgccggggaggtgcccataaagagcgcaaactccacgttttcccagtcgggtttgacatgcgggtttttatccagatcgcccatcaatgccccggagccggcccggtaagccagtccacagtaggcgccatgcgcgccgaaattcttgctgccgaagctatttagcgcaaaacgacgcagaaacgcatcgcggccttcgtcgctggtattcgtgaccagtaactgattggttttgggcccgaaactggggtgctttgcgtcaattggcgtatccggcgcatgaatagcgcgcagtccgtccacatgaccttcgccaaacagatcgccgccttccacgacttcttcaataagttgctcaaagctgatgcgctgccatttcccttcgccgcgtttacccacgcgtttcatcggttcaagcagtcgtagcggactgtacaggctttccagcagcgtggcgccgcgcgcgcaggcggttgagcgggcgtcaagaccgctttctcccgccagttgctccatggcttcgctaaaagggacggacgagtcaatcgggtgttcctgcgacaaggggtgatagggattgccggcgatgcgtatcactttgccatcggcattaacccgggcgcggataccgcactgtgtccaacagccgaagcattgcgtcatggcgatggtttgttgtggattttgctgccagtgtgtttgcgcctgcgcctccggaattaacgcattgccaaagatgcggtcgcgcgttaccttgccggacgtcccgtttaacaggccatcaattgcgcgtttcgccacatcacggtagctcagaccaaaagtgaccatcccaccgacggcgagaccgacttttagccactgacgacgggttaaattagccatgttgtaatctcctggtgagtccgttcagcgtttcacgaataataatcagtagcgctatccacaggccgaaggtgccgagaatagccagccagccatccgttccgcctggtaacgagtaagggttaaattgcgcgttgaacttggggacggtttgtacctgaatcaacaatgtccagcgcatcagccaacatagcgccagcgcgctgagaaccagcaggacgcgtcttagctgtgataacggatggcgtagcgccaggctacagaacagcagtgtgcatacccacagcgctacccagccgacagcgtaatatttggctgacagggcgacggtaatccactgacggattgccgtgccggaaagcgtatcgccgctaacccacatggccacaaccagccccagcgccgccagcgtccagatttgtccccacaatatttttggcagccttaccgagtcgcgtcgggcggcgacaatcatcagcgcgaagaacgcctgtaaggcgctaagaaacatcgccacggggaaggcgtagctaaaccagattgggcgcgccagcacaacggagacttcgcggccggtataaatcaacaggcccaccgcgcaaagcgcgctggctaacgccaaccatttagtgacgttgtaacttttattgaataatcgtttaatctgctgcgccaggaaccacagagcgagaaatccggtaaacagcggcaggaataacgctccccagggcatccacgaccagggcgtcggccaggcatagaaatgccagacgcgggcggtctggtgcagatccgccgtcagcgccagcggtgcggtaatcgcacaggtaatggcaatcagtaatgcccgattttcttctgttgcggcgtcttttttccgccagtgaagataacaggcaaacagtgcggcgcaggcggcaatgccaataaaaaagaaatattgtaccgcccacggcagccagctaatgtcctgcgggtgagccagcacttcttcaatgatgagtgaatgcgtcattcagacctcctgccaaagcgcgggctgcgcacggcccattaatggggtgacaaaggcgtcgtccagacccaggtagaaaacatggggcgacgtgccgttttccggctttaataccttgatagcgtcgcgatgctgatgaagcatggtggcgatgcggctatggggatctttgatatcgccaataatacgcgcgccgccgacgcaggactctacgcaagcgggtaacagtccggcttccagacgatggacgcaaaacgtgcatttatcggcagtttgcgtttcatgattgataaatcgggcgtcgtaaggacacgcctggacacaataggcgcagccgacgcagcgtttgttatccaccaccacaatgccatcttcccgctgaaaggtggcttgtaccgggcagaccggcacacagggggggttatcgcaatggttgcacagacgcggcaacagcacattcgtgacttcctgactaccttcacgctggacctggtattggttcaccgtcgtacgaaacgcgccttgcggcgtttggttttcaatagtgcaacttacggtacaggactgacagccgatacaacgccgcagatcgataagcatggcgtaacggtgtcggggagagccttcatgccgctccggcgaaaaaggaaatttcgcttcagccagcggaaccagcgaggcgccagcggtcaggacgccaagctgctggagaaattgccgtttactgctgtccatattgactcccgtccacattgccaacaatgaaacatttgtcacgatgttggttcatgtgtaatgaataaaaaatgtcgatgatttacagtgtaaaaatcgaggcggggtgcgctctattgtggttaaccacatacccggcttgttgttgatctaaaacaacataattgacagggatattggggtgagaggtaaaaccgtaaggcgcctggcggtgttggcggcagtagggctactttgtcatggcgcgtgggcagggacgtggaatatcggtattttggccatgcgcggcgaggcgtctacgcgtagccactggcaaccgttggcaaagacattaagccaacagcttccaggcgaaacctttcacatccagccgctggatctgcatcaaatgcaggaggccgttaaccagggaaccgtgcagtttgtgataaccaacccggcgcaatttgtccaactgaacagccatgcgccgctgcgctggttagcttccctgcgctccacgcgcgatgggaaagcggtgagtaatgttattggcagcgtgattttgacccggcgcgatagcggcatcaccacggcgcatgatctcatcggtaagaccgtcggcgcgattgatgctcaggcgtttggcggctatttattaggctataaagcgctcagcgacgcgggcttacgcccggagcgcgattttcatctccgttttaccggatttcctggcgatgccttagtctatatgctgcgcgaaaaagcggtgcaggcggcaattgtgccagtgtgcctgttagaaaatatggatcaggaaggattgattaataaaaaggactttatcgcgctgctttcccgaccgacgcccctgccttgcttaaccagtacgccgttatatcctgactggtcgttcgcggcgctacctgcggtaagcgatgcgctggcggatcgcgtaacgcgagcgctattcaacgcgcccgccgccgcgtcatttcactggggcgcgcctgcgtccaccagtcaggtggaagccttgctgcgtgatgttcgtcagcaccctcagcagcgtcgactgtggctggatgtcaaaagttggttaatccagcaccagctaatggtcggcggcgtgattctggcgttcttgttgctcacgctcaattatatttgggtcatgctgctggtgcgtcgacgtggaaagcaactggaacgtaatagcgtagttcttcatcagcatgagcgggcgctggaaaccgcccggcaaatgagcgtgttgggtgaaatgacctccgggtttgcccatgagcttaatcagccgctttccgcgattcgacattatgcccaggggtgcctgattcgactgcgcgctgcagatgaacagcatcccttgctgccggcgctggagcagattgaccagcaggcgcaacgcggtgcggatactctgcgtaacctgcgtcactgggtcagccaggcgcagggcaacccggtgctaaccgaagcgtggaaggccatagccattcgcgaggcgattgatcatgtctggcaattgttgcgtatggcgcaacagtttccgacagtgactctgcataccgaggttagcgctgcgctgcgcgtaacgctgccgtcagtgctgctggaacaggtgctggcgaatatcattcttaatgcggctcaggcgggcgccacccatttatggatcgttgctgaacgcactgaaaacggcatcagtattgttttacaggataacgccgggggaatcgatgaggcgctattacgtcaggcgtttcagccgtttatgaccacccgtaaagaggggatgggcttagggctggcgatttgccagcggctggtgcggtatgggcggggcgatatcagcatcaggaaccagaccgcgccggacggtctgtcgggaacggtggttacgatacatttcttacatgaaaatgggggcagggatggcgacaattcatctactggatgatgatacggcggtcactaacgcgtgcgcgtttttactggaaagtctgggatatgacgtaaaatgctggacgcagggggcggattttttggcgcaggccagtctgtatcaggccggggtcgtattactggatatgcgaatgccggtactggatgggcagggcgttcatgatgcgttgcgccagtgcggaagtaccctggcggttgtttttcttaccgggcatggcgatgtaccgatggccgtggagcagatgaaacgcggcgccgtcgattttctgcaaaaaccggtatcggtaaaaccgctacaggcggcgctggagcgtgcgctgacggtttcatcggcagcggtggcgcgtcgtgagattatactgtgttaccagcagttgacgccgaaagagcgtgagctggccagcctggtggcaaaaggatttatgaaccgtgaaattgcggaagcgatgaatatcgcggtgcgtaccgtagaggtgcaccgcgccagagtcatggaaaaaatgcaggccggtagcctggcggaactgattaggcgtttcgaaaaaatggcctcgccagagaccagaatacgaacaacgtatgagccatgaataagagctcgaattctcatgtttgacagcttatcactgatcagtgaattaatggcgatgacgcatcctcacgataatatccgggtaggcgcaatcactttcgtctctactccgttacaaagcgaggctgggtatttcccggcctttctgttatccgaaatccactgaaagcacagcggctggctgaggagataaataataaacgaggggctgtatgcacaaagcatcttctgttgagttaagaacgagtatcgagatggcacatagccttgctcaaattggaatcaggtttgtgccaataccagtagaaacagacgaagaagctagaggtgaatcacgacaaagcgtatcaaaaacgtatggagtagggctctaaactctgtataaaaagtttccagctagctgataacgggaaagaaacagagaagggcacaaatattgtgtactttaatgtgccctttaatttattgattggtggttgaattgtccgtaactttttgatttaagtgcaaatttctaataaattagaacactttcttaaatggtttcactgaaacgtgttcatagactcctgccgctacgtacgggtcagcatcggcccaagcctgagctgcttccagcgactcaaattcagcaataacggttgagccagtaaatcccgcagcc

SEQ ID NO: 48 - DNA, 4395 bp, synthetic construct
  misc_feature 1..4395: note = vector
  source 1..4395: mol_type = other DNA
gacctataaggaaaggccaaacaagaacacggttgcaaaaaccgtgcccttaaatattgaatttctattcagaacactttcttaaattgtcatttggcatattacgaacaattccgcgtaaaaacgttctgttacgctaaacccttatccagcaggctttcaaggatgtaaaccataacactctgcgaactagtgttacattgcgtgtagctttgagtgggcaactttgtgtacacttttgtgtacccaaaaacaaaaatgtgtacccattcaatgatcaccgacacaaagctcaggaaggcgctcggcaagaaaagagatgatatcgagattatttctgattcgcacgggcccatggctaattcccatgtcagccgttaagtgttcctgtgtcactgaaaattgctttgagaggctctaagggcttctcagtgcgttacatccctggcttgttgtccacaaccgttaaaccttaaaagctttaaaagccttatatattcttttttttcttataaaacttaaaaccttagaggctatttaagttgctgatttatattaattttattgttcaaacatgagagcttagtacgtgaaacatgagagcttagtacgttagccatgagagcttagtacgttagccatgagggtttagttcgttaaacatgagagcttagtacgttaaacatgagagcttagtacgtgaaacatgagagcttagtacgtactatcaacaggttgaactgctgatcttcagatcctctacgccggacgcatcgtggccggatcttgcggccgcaaaaattaaaaatgaagttttggaggcctcatttggtgacgaaataactaagcacttgtctcctgtttactcccctgagcttgaggggtcaacatgaaggtcattgatagcaggataataatacagtaaaacgctaaaccaataatccaaatccagccatcccaaattggtagtgaatgattataaataacagtaaacagtaatgggccaataacaccggttgcattggtaaggctcaccaataatccctgtaaagcaccttgctcatgactctttgtttggatagacatcactccctgtaatgcaggtaaagcgatcccaccaccagccaataaaattaaaacagggaaatctaaccaaccttcagatataaacgctaaaaaggcaaatgcactactatctgcaataaattcgagcagtactgccgttttttcgccccatttagtggctattcttcctgccacaaaggcttggaatactgagtgtaaaagaccaagacccgctaatgaaaagccaaccatcatgctattccatccaaaacgattttcggtaaatagcacccacaccgttgcgggaatttggcctatcaattgcgctgaaaaataaataatcaacaaaatgggcatcgttttaaataaagtgatgtacaccgaatttgattgcgtctcaacccctacttcggtatctgtattatcacgtgtatttttggtttcacggaaccaaaacataaccacaaggaaagtgacaatatttagcaacgcagcgataaaaaagggactatgcggtgaaatctctcctgcaaaaccaccaataataggccccgctattaaaccaagcccaaaacttgcccctaaccaaccgaaccacttcacgcgttgagaagctgaggtggtatcggcaatgaccgatgccgcgacagccccagtagctcctgtgatccctgaaagcaaacggcctaaatacagcatccaaagcgcacttgaaaaagccagcaataagtaatccagcgatgcgcctattaatgacaacaacagcactgggcgccgaccaaatcggtcagacatttttccaagccaaggagcaaagataacctgcattaacgcataaagtgcaagcaatacgccaaagtggttagcgatatcttccgaagcaataaattcacgtaataacgttggcaagactggcatgataaggccaatccccatggcatcgagtaacgtaattaccaatgcgatctttgtcgaactattcatttcacttttctctatcactgatagggagtgggaaaataactctatcaatgatagggtgtcaaatcgatggcccccgatggtagtgtggggtctccccatgcgagagtagggaactgccaggcatcaaataaaacgaaaggctcagtcgaaagactgggcctttcgttttatctgttgtttgtcggtgaacgctctcctgagtaggacaaatccgccgggagcggatttgaacgttgcgaagcaacggcccggagggtggcgggcaggacgcccgccataaactgccaggcatcaaattaagcagaaggccatcctgacggatggcctttttgcgtggccagtgccaagcttgcatgcctgcaggtcgactctagaggatccattccggggatccgtcgacctgcagttcgaagttcctattctctagaaagtataggaacttcagagcgcttttgaagctcacgctgccgcaagcactcagggcgcaagggctgctaaaggaagcggaacacgtagaaagccagtccgcagaaacggtgctgaccccggatgaatgtcagctactgggctatctggacaagggaaaacgcaagcgcaaagagaaagcaggtagcttgcagtgggcttacatggcgatagctagactgggcggttttatggacagcaagcgaaccggaattgccagctggggcgccctctggtaaggttgggaagccctgcaaagtaaactggatggctttcttgccgccaaggatctgatggcgcaggggatcaagatctgatcaagagacaggatgaggatcgtttcgcatgattgaacaagatggattgcacgcaggttctccggccgcttgggtggagaggctattcggctatgactgggcacaacagacaatcggctgctctgatgccgccgtgttccggctgtcagcgcaggggcgcccggttctttttgtcaagaccgacctgtccggtgccctgaatgaactgcaggacgaggcagcgcggctatcgtggctggccacgacgggcgttccttgcgcagctgtgctcgacgttgtcactgaagcgggaagggactggctgctattgggcgaagtgccggggcaggatctcctgtcatctcaccttgctcctgccgagaaagtatccatcatggctgatgcaatgcggcggctgcatacgcttgatccggctacctgcccattcgaccaccaagcgaaacatcgcatcgagcgagcacgtactcggatggaagccggtcttgtcgatcaggatgatctggacgaagagcatcaggggctcgcgccagccgaactgttcgccaggctcaaggcgcgcatgcccgacggcgaggatctcgtcgtgacccatggcgatgcctgcttgccgaatatcatggtggaaaatggccgcttttctggattcatcgactgtggccggctgggtgtggcggaccgctatcaggacatagcgttggctacccgtgatattgctgaagagcttggcggcgaatgggctgaccgcttcctcgtgctttacggtatcgccgctcccgattcgcagcgcatcgccttctatcgccttcttgacgagttcttctaataaggggatcttgaagttcctattccgaagttcctattctctagaaagtataggaacttcgaagcagctccagcctacagagctcgaattctcatgtttgacagcttatcactgatcagtgaattaatggcgatgacgcatcctcacgataatatccgggtaggcgcaatcactttcgtctctactccgttacaaagcgaggctgggtatttcccggcctttctgttatccgaaatccactgaaagcacagcggctggctgaggagataaataataaacgaggggctgtatgcacaaagcatcttctgttgagttaagaacgagtatcgagatggcacatagccttgctcaaattggaatcaggtttgtgccaataccagtagaaacagacgaagaagctagaggtgaatcacgacaaagcgtatcaaaaacgtatggagtagggctctaaactctgtataaaaagtttccagctagctgataacgggaaagaaacagagaagggcacaaatattgtgtactttaatgtgccctttaatttattgattggtggttgaattgtccgtaactttttgatttaagtgcaaatttctaataaattagaacactttcttaaatggtttcactgaaacgtgttcatagactcctgccgctacgtacgggtcagcatcggcccaagcctgagctgcttccagcgactcaaattcagcaataacggttgagccagtaaatcccgcagcc

SEQ ID NO: 49 - protein, 28 aa, synthetic construct
  REGION 1..28: note = linker
GSAGSAEAGSNWSHPQFEKGSAGSAAGS

SEQ ID NO: 50 - protein, 12 aa, synthetic construct
  REGION 1..12: note = linker
GSAGSAAGSGEF

SEQ ID NO: 51 - DNA, 84 bp, synthetic construct
  misc_feature 1..84: note = linker
  source 1..84: mol_type = other DNA
ggtagtgctggtagtgctgaagctggtagtaattggagtcatccacaatttgaaaaaggtagtgctggtagtgctgctggtagt

SEQ ID NO: 52 - DNA, 36 bp, synthetic construct
  misc_feature 1..36: note = linker
  source 1..36: mol_type = other DNA
ggtagtgctggtagtgctgctggtagtggtgaattt

SEQ ID NO: 53 - DNA, 3669 bp, Lactobacillus reuteri
  source 1..3669: mol_type = genomic DNA
atgctatcaagaaaaaattataaggaaactatacgaaaacagacacctacaaaacagtactatactattaagaaattaactgttggggttacttcggtattaattggtctatcctttatgggagaactagaaggggatagcgttcatgcggacacgatgacagcaagcagtgagtcaacaagtgttacgtcgacgactgctcaggatggtttaaaaaaatctccacaactctatttgcaagttactgatacaaataacccaagtacaccattaagtgcttcatccacagggactagtaagaatgttacctcatcagctgcggtacaagtgaagtccgctagtgatgaagaagatagtgattctacactagctaagggagaaaataaatttgctcggtcagcagtaaaagattcagtcactgatgggaaaacaagtacagcagaaattaatccggcaaaattaagcagtcctgctttaataacgcaactcaaccaatccttagctaagagcagtacgagtgatgcagcaaaagctaatgatgagttagaaattaaagcaacagatccgactaattatccaaactgtggcgatgtgtatgggccattatttgaattggatgctagcggacagcttgttaataaagatgaagttatatctcttaaagatatgtatattttccaaatattgaaattagtaaatacaaaagatagtgactttcaatatgtaatattaacaatgaatcgtaaagatactgcagataggtctgtatatctttttgtaactggaagcaattatagtaatgctgttgttgttaaagtaaagccaaatgatacttatgaattaagtaaaactggatatagtgttacttatacagaaccaacaactataaatggacattatgttgatggaactttttatgttacaggaagtacttacgatgatggttttataatgccagattggcaactgcagcaccttcagattatatatagtttaggaaattatgatccaagcaatactgacgcaacatcagtttgtgaaataatgccaagttatgaaaaggtaccggtaattaaatatagtggagtaccttcaaatattagccaacctaaggtttacattaccgggtttacgggtcaagagtttaacgttacagatattattaacaattataagaaagtttttaagggctactatcttcaaaatcctaatgtggcgtccatgggaactctttcccaatttgagaatggtggttattacttaaagacatattatgataatgatggtaatgttgactttaagggcttgtatcatcaaattgatgatcagggaacaatgagtgtgagtgttcttaatgcagataataaaacaattgttggacctgaaaatattcttgctggtaaatcgcataactttaactttaatggtcataactggattgcgcggaatccttatgtcactagttcagctcacgaagtcatattaaagtatgctaagttaggttcagttattcctgttgatgaaaacggaaataaaataaacgatggatggcaatatgttaatgatccagatgatgcttccaaagccactagcccatatgaaaaagcgccagttatcgatggttatgtagctgtaaatccagatgaaacgatcgttcttcctcataacttaagtagtgacacaaagatttattaccgaaagaggattaaagttacctatagtggtagtgacagcaagacctacgatggtaacccagctaacttcgagccaacgacagttcagtggagtggcttgaaaggactgaacacttcaaccttaacgtccgctgacttcacgtggaatactgcggataagaaggcaccaacggatgccggtaagtacacacttagtttgaatacgaccggagaagcagccttacgtaaggctaacccgaactatgatctcaagacaattagcggtagttacacctacacgattaatccactagggattgataaagttacctatagtggtagtgacagcaagacctacgatggtaacccagctaacttcgagccaacgacagttcagtggagtggcttgaaaggactgaacacttcaaccttaacgtccgctgacttcacgtggaatactgcggataagaaggcaccaacggatgccggtaagtacacacttagtttgaatacgaccggagaagcagccttacgtaaggctaacccgaactatgatctcaagacaattagcggtagttacacctacacgattaatccactagggattgataaagttacctatagtggtagtgacagcaagacctacgatggtaacccagctaacttcgagccaacgacagttcagtggagtggcttgaaaggactgaacacttcaaccttaacgtccgctgacttcacgtggaatactgcggataagaaggcaccaacggatgccggtaagtacacacttagtttgaatacgaccggagaagcagccttacgtaaggctaacccgaactatgatctcaagacaattagcggtagttacacctacacgattaatccactagggattgataaagttacctatagtggtagtgacagcaagacctacgatggtaacccagctaacttcgagccaacgacagttcagtggagtggcttgaaaggactgaacacttcaaccttaacgtccgctgacttcacgtggaatactgcggataagaaggcaccaacggatgccggtaagtacacacttagtttgaatacgaccggagaagcagccttacgtaaggctaacccgaactatgatctcaagacaattagcggtagttacacctacacgattaatccactagggattgataaagttacctatagtggtagtgacagcaagacctacgatggtaacccagctaacttcgagccaacgacagttcagtggagtggcttgaaaggactgaacacttcaaccttaacgtccgctgacttcacgtggaatactgcggataagaaggcaccaacggatgccggtaagtacacacttagtttgaatacgaccggagaagcagccttacgtaaggctaacccgaactatgatctcaagacaattagcggtagttacacctacacgattaatccactagggattgtgactgtaaattacaagggctatgataagaaagtctatgatggtcaacctggaacgattaatccgggtaaattaacgtggagtaagttgccagatggtacttcattgaagatgccaacatggagtatagatgatttcgcttgggaaacagctgatggcttagcaccaacggcagtaggaacttatcggattatcttgacggatgctggtaaggctgcactaaagaagattaatccaaattatgacttaagcagtattactggtgtctttacttatgaaattaagccagcacagacaccagaaatcttaggccaaacacctgagcaacaaccaggccaaaatactaatcaatcaggagctgaaaacggctttggttcttctacaaggcctaatgcatcaactaactccaatcttaatcaacttccacagactggtaatgagcattctaatactgcacttgctggtctagcattggctttcttgactgctatgcttggtttgggcaagaagcgtaaacatgattag

SEQ ID NO: 54 - DNA, 18 bp, synthetic construct
  misc_feature 1..18: note = Primer
  source 1..18: mol_type = other DNA
cggctaccacccaaggaa

SEQ ID NO: 55 - DNA, 18 bp, synthetic construct
  misc_feature 1..18: note = Primer
  source 1..18: mol_type = other DNA
gctggaattaccgcggct

SEQ ID NO: 56 - DNA, 21 bp, synthetic construct
  misc_feature 1..21: note = Primer
  source 1..21: mol_type = other DNA
accgtgaatcttggctgtaac

SEQ ID NO: 57 - DNA, 21 bp, synthetic construct
  misc_feature 1..21: note = Primer
  source 1..21: mol_type = other DNA
gcagcaaatcgcttgggatta

SEQ ID NO: 58 - DNA, 20 bp, synthetic construct
  misc_feature 1..20: note = Primer
  source 1..20: mol_type = other DNA
tgtcagtcatcgcccatgtg

SEQ ID NO: 59 - DNA, 21 bp, synthetic construct
  misc_feature 1..21: note = Primer
  source 1..21: mol_type = other DNA
catccttgcgagtgtcagtga

SEQ ID NO: 60 - DNA, 24 bp, synthetic construct
  misc_feature 1..24: note = Primer
  source 1..24: mol_type = other DNA
catcttctcaaaattcgagtgaca

SEQ ID NO: 61 - DNA, 23 bp, synthetic construct
  misc_feature 1..23: note = Primer
  source 1..23: mol_type = other DNA
tgggagtagacaaggtacaaccc

SEQ ID NO: 62 - DNA, 23 bp, synthetic construct
  misc_feature 1..23: note = Primer
  source 1..23: mol_type = other DNA
tcaagtggcatagatgtggaaga

SEQ ID NO: 63 - DNA, 21 bp, synthetic construct
  misc_feature 1..21: note = Primer
  source 1..21: mol_type = other DNA
tggctctgcaggattttcatg

SEQ ID NO: 64 - DNA, 20 bp, synthetic construct
  misc_feature 1..20: note = Primer
  source 1..20: mol_type = other DNA
agggccctttgctatggtgt

SEQ ID NO: 65 - DNA, 20 bp, synthetic construct
  misc_feature 1..20: note = Primer
  source 1..20: mol_type = other DNA
tggccacagttttcagggat

SEQ ID NO: 66 - DNA, 20 bp, synthetic construct
  misc_feature 1..20: note = Primer
  source 1..20: mol_type = other DNA
agcttccttgtgcaagtgtc

SEQ ID NO: 67 - DNA, 20 bp, synthetic construct
  misc_feature 1..20: note = Primer
  source 1..20: mol_type = other DNA
cccttcatcttttggggtcc

SEQ ID NO: 68 - DNA, 20 bp, synthetic construct
  misc_feature 1..20: note = Primer
  source 1..20: mol_type = other DNA
tccctctgtgatctgggaag

SEQ ID NO: 69 - DNA, 20 bp, synthetic construct
  misc_feature 1..20: note = Primer
  source 1..20: mol_type = other DNA
ctcgaccctgaaagtgaagg

SEQ ID NO: 70 - DNA, 22 bp, synthetic construct
  misc_feature 1..22: note = Primer
  source 1..22: mol_type = other DNA
cccgtataaccatcaccatcat

SEQ ID NO: 71 - DNA, 21 bp, synthetic construct
  misc_feature 1..21: note = Primer
  source 1..21: mol_type = other DNA
ggcatctttcttggcaacttc

SEQ ID NO: 72 - DNA, 17 bp, synthetic construct
  misc_feature 1..17: note = Primer
  source 1..17: mol_type = other DNA
gccagatcccgaaacca

SEQ ID NO: 73 - DNA, 20 bp, synthetic construct
  misc_feature 1..20: note = Primer
  source 1..20: mol_type = other DNA
tataggagtctcggcagtca